European Patent Application EP 4 248 979 A2, published September 27, 2023. Title: PD-1 HOMING ENDONUCLEASE VARIANTS, COMPOSITIONS, AND METHODS OF USE. Applicant: 2seventy bio, Inc. The sequence listing filed with the application follows.

SEQUENCE LISTING (123 sequences)

SEQ ID NO: 1 - protein, 303 aa, Ophiostoma novo-ulmi
  source 1..303: note = subsp. americana (mitochondrion)
MAYMSRRESINPWILTGFADAEGSFLLRIRNNNKSSVGYSTELGFQITLHNKDKSILENIQSTWKVGVIANSGDNAVSLKVTRFEDLKVIIDHFEKYPLITQKLGDYMLFKQAFCVMENKEHLKINGIKELVRIKAKLNWGLTDELKKAFPEIISKERSLINKNIPNFKWLAGFTSGEGCFFVNLIKSKSKLGVQVQLVFSITQHIKDKNLMNSLITYLGCGYIKEKNKSEFSWLDFVVTKFSDINDKIIPVFQENTLIGVKLEDFEDWCKVAKLIEEKKHLTESGLDEIKKIKLNMNKGRVF

SEQ ID NO: 2 - protein, 303 aa, Ophiostoma novo-ulmi
  source 1..303: note = subsp. americana (mitochondrion)
MAYMSRRESINPWILTGFADAEGSFLLRIRNNNKSSVGYSTELGFQITLHNKDKSILENIQSTWKVGVIANSGDNAVSLKVTRFEDLKVIIDHFEKYPLITQKLGDYKLFKQAFSVMENKEHLKENGIKELVRIKAKLNWGLTDELKKAFPENISKERSLINKNIPNFKWLAGFTSGEGCFFVNLIKSKSKLGVQVQLVFSITQHIKDKNLMNSLITYLGCGYIKEKNKSEFSWLDFVVTKFSDINDKIIPVFQENTLIGVKLEDFEDWCKVAKLIEEKKHLTESGLDEIKKIKLNMNKGRVF

SEQ ID NO: 3 - protein, 303 aa, Ophiostoma novo-ulmi
  MOD_RES 1..3: note = Any amino acid or absent
  source 1..303: note = subsp. americana (mitochondrion)
XXXMSRRESINPWILTGFADAEGSFLLRIRNNNKSSVGYSTELGFQITLHNKDKSILENIQSTWKVGVIANSGDNAVSLKVTRFEDLKVIIDHFEKYPLITQKLGDYKLFKQAFSVMENKEHLKENGIKELVRIKAKLNWGLTDELKKAFPENISKERSLINKNIPNFKWLAGFTSGEGCFFVNLIKSKSKLGVQVQLVFSITQHIKDKNLMNSLITYLGCGYIKEKNKSEFSWLDFVVTKFSDINDKIIPVFQENTLIGVKLEDFEDWCKVAKLIEEKKHLTESGLDEIKKIKLNMNKGRVF

SEQ ID NO: 4 - protein, 303 aa, Ophiostoma novo-ulmi
  MOD_RES 1..4: note = Any amino acid or absent
  MOD_RES 302..303: note = Any amino acid or absent
  source 1..303: note = subsp. americana (mitochondrion)
XXXXSRRESINPWILTGFADAEGSFLLRIRNNNKSSVGYSTELGFQITLHNKDKSILENIQSTWKVGVIANSGDNAVSLKVTRFEDLKVIIDHFEKYPLITQKLGDYKLFKQAFSVMENKEHLKENGIKELVRIKAKLNWGLTDELKKAFPENISKERSLINKNIPNFKWLAGFTSGEGCFFVNLIKSKSKLGVQVQLVFSITQHIKDKNLMNSLITYLGCGYIKEKNKSEFSWLDFVVTKFSDINDKIIPVFQENTLIGVKLEDFEDWCKVAKLIEEKKHLTESGLDEIKKIKLNMNKGRXX

SEQ ID NO: 5 - protein, 303 aa, Ophiostoma novo-ulmi
  MOD_RES 1..8: note = Any amino acid or absent
  MOD_RES 302..303: note = Any amino acid or absent
  source 1..303: note = subsp. americana (mitochondrion)
XXXXXXXXSINPWILTGFADAEGSFLLRIRNNNKSSVGYSTELGFQITLHNKDKSILENIQSTWKVGVIANSGDNAVSLKVTRFEDLKVIIDHFEKYPLITQKLGDYKLFKQAFSVMENKEHLKENGIKELVRIKAKLNWGLTDELKKAFPENISKERSLINKNIPNFKWLAGFTSGEGCFFVNLIKSKSKLGVQVQLVFSITQHIKDKNLMNSLITYLGCGYIKEKNKSEFSWLDFVVTKFSDINDKIIPVFQENTLIGVKLEDFEDWCKVAKLIEEKKHLTESGLDEIKKIKLNMNKGRXX

SEQ ID NO: 6 - protein, 303 aa, synthetic construct
  REGION 1..303: note = Synthesized I-OnuI variant PD-1.ITSM.ex5_RD1_CV3-08
  MOD_RES 1..4: note = Any amino acid or absent
  MOD_RES 302..303: note = Any amino acid or absent
XXXXSRRESINPWILTGFADAEGSFQLEIRNVNPNIPRYKTRLRFEIDLHNKDKSILENIQSTWKVGKIYNQGDSYVKLRVTRFEDLKVIIDHFEKYPLITQKLGDYKLFKQAFSVMENKEHLKENGIKELVRIKAKMNWGLNDELKKAFPENISKERPLINKNIPNLKWLAGFTSGEGHFGVILAKRRPASPVQVRLRFAIGQHIRDKNLMNSLITYLGCGRIREKNISEKSWLEFEVTKFSDINDKIIPVFQENTLIGVKLEDFEDWCKVAKLIEEKKHLTESGLDEIKKIKLNMNKGRXX

SEQ ID NO: 7 - protein, 303 aa, synthetic construct
  REGION 1..303: note = Synthesized I-OnuI variant PD-1.ITSM.ex5_RD2_73
  MOD_RES 1..4: note = Any amino acid or absent
  MOD_RES 302..303: note = Any amino acid or absent
XXXXSRRESINPWILTGFADAEGSFQLEIRNVNPNIPRYRTRLRFEIDLHNKDKSILEDIQSTWKVGKIYNRGDSYVKLRVTRFEDLKVIIDHFEKYPLITQKLGDYKLFKQAFSVMENKEHLKENGIKELVRIKAKMNWGLNDELKKAFPENISKERPLINKNIPNLKWLAGFTSGEGHFGVILAKRRPASPVQVRLRFAIGQHIRDKNLMNSLITYLGCGRTREKNISEKSWLEFEVTKFSDINDKIIPVFQENTLIGVKLEDFEDWCKVAKLIEEKKHLTESGLDEIKKIKLNMNKGRXX

SEQ ID NO: 8 - protein, 303 aa, synthetic construct
  REGION 1..303: note = Synthesized I-OnuI variant PD-1.ITSM.ex5_RD3_03
  MOD_RES 1..4: note = Any amino acid or absent
  MOD_RES 302..303: note = Any amino acid or absent
XXXXSRRESINPWILTGFADAEGSFQLEIRNVNPNIPRYRTRLRFEIDLHNKDKSILEDIQSTWKVGKIYNQGDSYVKLRVTRFEDLKVIIDHFEKYPLITQKLGDYKLFKQAFSVMENKEHLKENGIKELVRIKAKMNWGLNDELKKAFPENISKERPLINKNIPNLKWLAGFTSGDGHFGVILAKRRPASPVQVRLRFAIGQHIRDKNLMNSLITYLGCGRTREKNISEKSWLEFEVTKFSDINDKIIPVFQENTLIGVKLEDFEDWCKVAKLIEEKKHLTESGLDEIKKIKLNMNKGRXX

SEQ ID NO: 9 - protein, 303 aa, synthetic construct
  REGION 1..303: note = Synthesized I-OnuI variant PD-1.ITSM.ex5_RD4_CV23
  MOD_RES 1..4: note = Any amino acid or absent
  MOD_RES 302..303: note = Any amino acid or absent
XXXXSRRESINPWILTGFADAEGSFQLEIRNVNPNIPRYRTRLRFEIDLHNKDKSILEDIQSTWKVGKIYNQGDSYVKLRVTRFEDLKVIIDHFEKYPLITQKLGDYKLFKQAFSVMENKEHLKENGIKELVRIKAKMNWGLNDELKKAFPENISKERPLINKNIPNLKWLAGFTSGDGHFGVILAKRRPASPVQVRLRFAIGQHIRDKNLMNSLITYLGCGRIREKNKSEKSWLEFEVTKFSDINDKIIPVFQENTLIGVKLEDFEDWCKVAKLIEEKKHLTESGLDEIKKIKLNMNKGRXX

SEQ ID NO: 10 - protein, 303 aa, synthetic construct
  REGION 1..303: note = Synthesized I-OnuI variant PD-1.ITSM.ex5_RD5_CV23MK
  MOD_RES 1..4: note = Any amino acid or absent
  MOD_RES 302..303: note = Any amino acid or absent
XXXXSRRESINPWILTGFADAEGSFQLEIRNVNPNIPRYRTRLRFEIDLHNKDKSILEDIQSTWKVGKIYNQGDSYVKLRVTRFEDLKVIIDHFEKYPLITQKLGDYKLFKQAFSVMENKEHLKENGIKELVRIKAKMNWGLNDELKKAFPENISKERPLINKNIPNLKWLAGFTSGDGHFGVILAKRRPASPVQVRLRFMIGQHIKDKNLMNSLITYLGCGRIREKNKSEKSWLEFEVTKFSDINDKIIPVFQENTLIGVKLEDFEDWCKVAKLIEEKKHLTESGLDEIKKIKLNMNKGRXX

SEQ ID NO: 11 - protein, 303 aa, synthetic construct
  REGION 1..303: note = Synthesized I-OnuI variant PD-1.ile3.exon1_RD1_B1
  MOD_RES 1..4: note = Any amino acid or absent
  MOD_RES 302..303: note = Any amino acid or absent
XXXXSRRESINPWILTGFADAEGSFGLSILNRNRGTARYHTRLSFAIVLHNKDKSILENIQSTWKVGIITNDGDRYVRLRVTRFEDLKVIIDHFEKYPLVTQKLGDYKLFKQAFSVMENKEHLKENGIKELVRIKAKMNWGLNDELKKAFPENISKERPLINKNIPNFKWLAGFTSGDGSFFVRLRKSNVNARVRVQLVFEISQHIRDKNLMNSLITYLGCGHIYEGNKSERSWLQFRVEKFSDINDKIIPVFQENTLIGVKLEDFEDWCKVAKLIEEKKHLTESGLDEIKKIKLNMNKGRXX

SEQ ID NO: 12 - protein, 303 aa, synthetic construct
  REGION 1..303: note = Synthesized I-OnuI variant PD-1.ile3.exon1_RD2_B1H8
  MOD_RES 1..4: note = Any amino acid or absent
  MOD_RES 302..303: note = Any amino acid or absent
XXXXSRRESINPWILTGFADAEGSFGLSILNRNRGTARYHTRLSFTIVLHNKDKSILENIQSTWKVGIITNDGDRYVRLCVTRFEDLKVIIDHFEKYPLVTQKLGDYKLFKQAFSVMENKEHLKENGIKELARIKAKMNWGLNDELKKAFPENIGKERPLINKNIPNFKWLAGFTSGDGSFFVRLRKSNVNARVRVQLVFEISQHIRDKNLMNSLITYLGCGHIYEGNKSERSWLQFRVEKFSDINDKIIPVFQENTLIGVKLEDFEDWCKVAKLIEEKKHLTESGLDEIKKIKLNMNKGRXX

SEQ ID NO: 13 - protein, 303 aa, synthetic construct
  REGION 1..303: note = Synthesized I-OnuI variant PD-1.IgV.exon2_RD1_G5
  MOD_RES 1..4: note = Any amino acid or absent
  MOD_RES 302..303: note = Any amino acid or absent
XXXXSRRESINPWILTGFADAEGSFQLYISNVNNNRSRYRARLRFAIELHNKDKSILENIQSTWKVGVINNIGDTSVRLSVGRFEDLKVIIDHFEKYPLITQKLGDYKLFKQAFSVMENKEHLKENGIKELVRIKAKMNWGLNDELKKAFPENISKERPLINKNIPNLKWLAGFTSGDGNFYVHLKKSGRTTRVYVQLRFSIAQHIRDKNLMNSLITYLGCGYINEWNASERSALEFRVTKFSDINDKIIPVFQENTLIGVKLEDFEDWCKVAKLIEEKKHLTESGLDEIKKIKLNMNKGRXX

SEQ ID NO: 14 - protein, 303 aa, synthetic construct
  REGION 1..303: note = Synthesized I-OnuI variant PD-1.IgV.exon2_RD1_PS3
  MOD_RES 1..4: note = Any amino acid or absent
  MOD_RES 302..303: note = Any amino acid or absent
XXXXSRRESINPWILTGFADAEGCFLLHIRNLNRTSTKYRTRLSFEIELHNKDKSILENIQSTWKVGIINNIGNRRVRLSVRRFEDLKVIIDHFEKYPLITQKLGDYKLFKQAFSLMENKEHLKENGIKELVRIKAKMNWGLNDELKKAFPENISKERPLINKNIPNLKWLAGFTSGDGNFYVHLKKSGRTTRVYVQLRFSISQHIRDKNLMNSLITYLGCGYITESNPSERSDLEFRVTKFSDINDKIIPVFQENTLIGVKLEDFEDWCKVAKLIEEKKHLTESGLDEIKKIKLNMNKGRXX

SEQ ID NO: 15 - protein, 870 aa, synthetic construct
  REGION 1..870: note = Synthesized megaTAL PD-1.ITSM.ex5_RD1_CV3-08
MGSAPPKKKRKVVDLRTLGYSQQQQEKIKPKVRSTVAQHHEALVGHGFTHAHIVALSQHPAALGTVAVTYQHIITALPEATHEDIVGVGKQWSGARALEALLTDAGELRGPPLQLDTGQLVKIAKRGGVTAMEAVHASRNALTGAPLNLTPDQVVAIASNGGGKQALETVQRLLPVLCQDHGLTPDQVVAIASHDGGKQALETVQRLLPVLCQDHGLTPDQVVAIASNGGKQALETVQRLLPVLCQDHGLTPDQVVAIASNNGGKQALETVQRLLPVLCQDHGLTPDQVVAIASHDGGKQALETVQRLLPVLCQDHGLTPDQVVAIASNGGGKQALETVQRLLPVLCQDHGLTPDQVVAIASNIGGKQALETVQRLLPVLCQDHGLTPDQVVAIASNNGGKQALETVQRLLPVLCQDHGLTPDQVVAIASNNGGKQALETVQRLLPVLCQDHGLTPDQVVAIASNIGGKQALETVQRLLPVLCQDHGLTPDQVVAIASNIGGKQALESIVAQLSRPDPALAALTNDHLVALACLGGRPAMDAVKKGLPHAPELIRRVNRRIGERTSHRVAISRSRRESINPWILTGFADAEGSFQLEIRNVNPNIPRYKTRLRFEIDLHNKDKSILENIQSTWKVGKIYNQGDSYVKLRVTRFEDLKVIIDHFEKYPLITQKLGDYKLFKQAFSVMENKEHLKENGIKELVRIKAKMNWGLNDELKKAFPENISKERPLINKNIPNLKWLAGFTSGEGHFGVILAKRRPASPVQVRLRFAIGQHIRDKNLMNSLITYLGCGRIREKNISEKSWLEFEVTKFSDINDKIIPVFQENTLIGVKLEDFEDWCKVAKLIEEKKHLTESGLDEIKKIKLNMNKGR

SEQ ID NO: 16 - protein, 870 aa, synthetic construct
  REGION 1..870: note = Synthesized megaTAL PD-1.ITSM.ex5_RD2_73
MGSAPPKKKRKVVDLRTLGYSQQQQEKIKPKVRSTVAQHHEALVGHGFTHAHIVALSQHPAALGTVAVTYQHIITALPEATHEDIVGVGKQWSGARALEALLTDAGELRGPPLQLDTGQLVKIAKRGGVTAMEAVHASRNALTGAPLNLTPDQVVAIASNGGGKQALETVQRLLPVLCQDHGLTPDQVVAIASHDGGKQALETVQRLLPVLCQDHGLTPDQVVAIASNGGKQALETVQRLLPVLCQDHGLTPDQVVAIASNNGGKQALETVQRLLPVLCQDHGLTPDQVVAIASHDGGKQALETVQRLLPVLCQDHGLTPDQVVAIASNGGGKQALETVQRLLPVLCQDHGLTPDQVVAIASNIGGKQALETVQRLLPVLCQDHGLTPDQVVAIASNNGGKQALETVQRLLPVLCQDHGLTPDQVVAIASNNGGKQALETVQRLLPVLCQDHGLTPDQVVAIASNIGGKQALETVQRLLPVLCQDHGLTPDQVVAIASNIGGKQALESIVAQLSRPDPALAALTNDHLVALACLGGRPAMDAVKKGLPHAPELIRRVNRRIGERTSHRVAISRSRRESINPWILTGFADAEGSFQLEIRNVNPNIPRYRTRLRFEIDLHNKDKSILEDIQSTWKVGKIYNRGDSYVKLRVTRFEDLKVIIDHFEKYPLITQKLGDYKLFKQAFSVMENKEHLKENGIKELVRIKAKMNWGLNDELKKAFPENISKERPLINKNIPNLKWLAGFTSGEGHFGVILAKRRPASPVQVRLRFAIGQHIRDKNLMNSLITYLGCGRTREKNISEKSWLEFEVTKFSDINDKIIPVFQENTLIGVKLEDFEDWCKVAKLIEEKKHLTESGLDEIKKIKLNMNKGR

SEQ ID NO: 17 - protein, 870 aa, synthetic construct
  REGION 1..870: note = Synthesized megaTAL PD-1.ITSM.ex5_RD3_03
MGSAPPKKKRKVVDLRTLGYSQQQQEKIKPKVRSTVAQHHEALVGHGFTHAHIVALSQHPAALGTVAVTYQHIITALPEATHEDIVGVGKQWSGARALEALLTDAGELRGPPLQLDTGQLVKIAKRGGVTAMEAVHASRNALTGAPLNLTPDQVVAIASNGGGKQALETVQRLLPVLCQDHGLTPDQVVAIASHDGGKQALETVQRLLPVLCQDHGLTPDQVVAIASNGGKQALETVQRLLPVLCQDHGLTPDQVVAIASNNGGKQALETVQRLLPVLCQDHGLTPDQVVAIASHDGGKQALETVQRLLPVLCQDHGLTPDQVVAIASNGGGKQALETVQRLLPVLCQDHGLTPDQVVAIASNIGGKQALETVQRLLPVLCQDHGLTPDQVVAIASNNGGKQALETVQRLLPVLCQDHGLTPDQVVAIASNNGGKQALETVQRLLPVLCQDHGLTPDQVVAIASNIGGKQALETVQRLLPVLCQDHGLTPDQVVAIASNIGGKQALESIVAQLSRPDPALAALTNDHLVALACLGGRPAMDAVKKGLPHAPELIRRVNRRIGERTSHRVAISRSRRESINPWILTGFADAEGSFQLEIRNVNPNIPRYRTRLRFEIDLHNKDKSILEDIQSTWKVGKIYNQGDSYVKLRVTRFEDLKVIIDHFEKYPLITQKLGDYKLFKQAFSVMENKEHLKENGIKELVRIKAKMNWGLNDELKKAFPENISKERPLINKNIPNLKWLAGFTSGDGHFGVILAKRRPASPVQVRLRFAIGQHIRDKNLMNSLITYLGCGRTREKNISEKSWLEFEVTKFSDINDKIIPVFQENTLIGVKLEDFEDWCKVAKLIEEKKHLTESGLDEIKKIKLNMNKGR

SEQ ID NO: 18 - protein, 870 aa, synthetic construct
  REGION 1..870: note = Synthesized megaTAL PD-1.ITSM.ex5_RD4_CV23
MGSAPPKKKRKVVDLRTLGYSQQQQEKIKPKVRSTVAQHHEALVGHGFTHAHIVALSQHPAALGTVAVTYQHIITALPEATHEDIVGVGKQWSGARALEALLTDAGELRGPPLQLDTGQLVKIAKRGGVTAMEAVHASRNALTGAPLNLTPDQVVAIASNGGGKQALETVQRLLPVLCQDHGLTPDQVVAIASHDGGKQALETVQRLLPVLCQDHGLTPDQVVAIASNGGKQALETVQRLLPVLCQDHGLTPDQVVAIASNNGGKQALETVQRLLPVLCQDHGLTPDQVVAIASHDGGKQALETVQRLLPVLCQDHGLTPDQVVAIASNGGGKQALETVQRLLPVLCQDHGLTPDQVVAIASNIGGKQALETVQRLLPVLCQDHGLTPDQVVAIASNNGGKQALETVQRLLPVLCQDHGLTPDQVVAIASNNGGKQALETVQRLLPVLCQDHGLTPDQVVAIASNIGGKQALETVQRLLPVLCQDHGLTPDQVVAIASNIGGKQALESIVAQLSRPDPALAALTNDHLVALACLGGRPAMDAVKKGLPHAPELIRRVNRRIGERTSHRVAISRSRRESINPWILTGFADAEGSFQLEIRNVNPNIPRYRTRLRFEIDLHNKDKSILEDIQSTWKVGKIYNQGDSYVKLRVTRFEDLKVIIDHFEKYPLITQKLGDYKLFKQAFSVMENKEHLKENGIKELVRIKAKMNWGLNDELKKAFPENISKERPLINKNIPNLKWLAGFTSGDGHFGVILAKRRPASPVQVRLRFAIGQHIRDKNLMNSLITYLGCGRIREKNKSEKSWLEFEVTKFSDINDKIIPVFQENTLIGVKLEDFEDWCKVAKLIEEKKHLTESGLDEIKKIKLNMNKGR

SEQ ID NO: 19 - protein, 870 aa, synthetic construct
  REGION 1..870: note = Synthesized megaTAL PD-1.ITSM.ex5_RD5_CV23MK
MGSAPPKKKRKVVDLRTLGYSQQQQEKIKPKVRSTVAQHHEALVGHGFTHAHIVALSQHPAALGTVAVTYQHIITALPEATHEDIVGVGKQWSGARALEALLTDAGELRGPPLQLDTGQLVKIAKRGGVTAMEAVHASRNALTGAPLNLTPDQVVAIASNGGGKQALETVQRLLPVLCQDHGLTPDQVVAIASHDGGKQALETVQRLLPVLCQDHGLTPDQVVAIASNGGKQALETVQRLLPVLCQDHGLTPDQVVAIASNNGGKQALETVQRLLPVLCQDHGLTPDQVVAIASHDGGKQALETVQRLLPVLCQDHGLTPDQVVAIASNGGGKQALETVQRLLPVLCQDHGLTPDQVVAIASNIGGKQALETVQRLLPVLCQDHGLTPDQVVAIASNNGGKQALETVQRLLPVLCQDHGLTPDQVVAIASNNGGKQALETVQRLLPVLCQDHGLTPDQVVAIASNIGGKQALETVQRLLPVLCQDHGLTPDQVVAIASNIGGKQALESIVAQLSRPDPALAALTNDHLVALACLGGRPAMDAVKKGLPHAPELIRRVNRRIGERTSHRVAISRSRRESINPWILTGFADAEGSFQLEIRNVNPNIPRYRTRLRFEIDLHNKDKSILEDIQSTWKVGKIYNQGDSYVKLRVTRFEDLKVIIDHFEKYPLITQKLGDYKLFKQAFSVMENKEHLKENGIKELVRIKAKMNWGLNDELKKAFPENISKERPLINKNIPNLKWLAGFTSGDGHFGVILAKRRPASPVQVRLRFMIGQHIKDKNLMNSLITYLGCGRIREKNKSEKSWLEFEVTKFSDINDKIIPVFQENTLIGVKLEDFEDWCKVAKLIEEKKHLTESGLDEIKKIKLNMNKGR

SEQ ID NO: 20 - protein, 841 aa, synthetic construct
  REGION 1..841: note = Synthesized megaTAL PD-1.ile3.exon1_RD1 B1
MGSAPPKKKRKVVDLRTLGYSQQQQEKIKPKVRSTVAQHHEALVGHGFTHAHIVALSQHPAALGTVAVTYQHIITALPEATHEDIVGVGKQWSGARALEALLTDAGELRGPPLQLDTGQLVKIAKRGGVTAMEAVHASRNALTGAPLNLTPDQVVAIASNNGGKQALETVQRLLPVLCQDHGLTPDQVVAIASNNGGKQALETVQRLLPVLCQDHGLTPDQVVAIASNGGGKQALETVQRLLPVLCQDHGLTPDQVVAIASNNGGKQALETVQRLLPVLCQDHGLTPDQVVAIASNNGGKQALETVQRLLPVLCQDHGLTPDQVVAIASNNGGKQALETVQRLLPVLCQDHGLTPDQVVAIASNNGGKQALETVQRLLPVLCQDHGLTPDQVVAIASHDGGKQALETVQRLLPVLCQDHGLTPDQVVAIASNGGGKQALETVQRLLPVLCQDHGLTPDQVVAIASNNGGKQALESIVAQLSRPDPALAALTNDHLVALACLGGRPAMDAVKKGLPHAPELIRRVNRRIGERTSHRVAISRVGGSSRRESINPWILTGFADAEGSFGLSILNRNRGTARYHTRLSFAIVLHNKDKSILENIQSTWKVGIITNDGDRYVRLRVTRFEDLKVIIDHFEKYPLVTQKLGDYKLFKQAFSVMENKEHLKENGIKELVRIKAKMNWGLNDELKKAFPENISKERPLINKNIPNFKWLAGFTSGDGSFFVRLRKSNVNARVRVQLVFEISQHIRDKNLMNSLITYLGCGHIYEGNKSERSWLQFRVEKFSDINDKIIPVFQENTLIGVKLEDFEDWCKVAKLIEEKKHLTESGLDEIKKIKLNMNKGR

SEQ ID NO: 21 - protein, 841 aa, synthetic construct
  REGION 1..841: note = Synthesized megaTAL PD-1.ile3.exon1_RD2_B1H8
MGSAPPKKKRKVVDLRTLGYSQQQQEKIKPKVRSTVAQHHEALVGHGFTHAHIVALSQHPAALGTVAVTYQHIITALPEATHEDIVGVGKQWSGARALEALLTDAGELRGPPLQLDTGQLVKIAKRGGVTAMEAVHASRNALTGAPLNLTPDQVVAIASNNGGKQALETVQRLLPVLCQDHGLTPDQVVAIASNNGGKQALETVQRLLPVLCQDHGLTPDQVVAIASNGGGKQALETVQRLLPVLCQDHGLTPDQVVAIASNNGGKQALETVQRLLPVLCQDHGLTPDQVVAIASNNGGKQALETVQRLLPVLCQDHGLTPDQVVAIASNNGGKQALETVQRLLPVLCQDHGLTPDQVVAIASNNGGKQALETVQRLLPVLCQDHGLTPDQVVAIASHDGGKQALETVQRLLPVLCQDHGLTPDQVVAIASNGGGKQALETVQRLLPVLCQDHGLTPDQVVAIASNNGGKQALESIVAQLSRPDPALAALTNDHLVALACLGGRPAMDAVKKGLPHAPELIRRVNRRIGERTSHRVAISRVGGSSRRESINPWILTGFADAEGSFGLSILNRNRGTARYHTRLSFTIVLHNKDKSILENIQSTWKVGIITNDGDRYVRLCVTRFEDLKVIIDHFEKYPLVTQKLGDYKLFKQAFSVMENKEHLKENGIKELARIKAKMNWGLNDELKKAFPENIGKERPLINKNIPNFKWLAGFTSGDGSFFVRLRKSNVNARVRVQLVFEISQHIRDKNLMNSLITYLGCGHIYEGNKSERSWLQFRVEKFSDINDKIIPVFQENTLIGVKLEDFEDWCKVAKLIEEKKHLTESGLDEIKKIKLNMNKGR

SEQ ID NO: 22 - protein, 909 aa, synthetic construct
  REGION 1..909: note = Synthesized megaTAL PD-1.IgV.exon2_RD1_G5
MGSAPPKKKRKVVDLRTLGYSQQQQEKIKPKVRSTVAQHHEALVGHGFTHAHIVALSQHPAALGTVAVTYQHIITALPEATHEDIVGVGKQWSGARALEALLTDAGELRGPPLQLDTGQLVKIAKRGGVTAMEAVHASRNALTGAPLNLTPDQVVAIASNNGGKQALETVQRLLPVLCQDHGLTPDQVVAIASNGGGKQALETVQRLLPVLCQDHGLTPDQVVAIASHDGGKQALETVQRLLPVLCQDHGLTPDQVVAIASNIGGKQALETVQRLLPVLCQDHGLTPDQVVAIASHDGGKQALETVQRLLPVLCQDHGLTPDQVVAIASNIGGKQALETVQRLLPVLCQDHGLTPDQVVAIASHDGGKQALETVQRLLPVLCQDHGLTPDQVVAIASNIGGKQALETVQRLLPVLCQDHGLTPDQVVAIASNIGGKQALETVQRLLPVLCQDHGLTPDQVVAIASHDGGKQALETVQRLLPVLCQDHGLTPDQVVAIASNGGGKQALETVQRLLPVLCQDHGLTPDQVVAIASNNGGKQALESIVAQLSRPDPALAALTNDHLVALACLGGRPAMDAVKKGLPHAPELIRRVNRRIGERTSHRVAISRVGGSSRRESINPWILTGFADAEGSFQLYISNVNNNRSRYRARLRFAIELHNKDKSILENIQSTWKVGVINNIGDTSVRLSVGRFEDLKVIIDHFEKYPLITQKLGDYKLFKQAFSVMENKEHLKENGIKELVRIKAKMNWGLNDELKKAFPENISKERPLINKNIPNLKWLAGFTSGDGNFYVHLKKSGRTTRVYVQLRFSIAQHIRDKNLMNSLITYLGCGYINEWNASERSALEFRVTKFSDINDKIIPVFQENTLIGVKLEDFEDWCKVAKLIEEKKHLTESGLDEIKKIKLNMNKGR

SEQ ID NO: 23 - protein, 909 aa, synthetic construct
  REGION 1..909: note = Synthesized megaTAL PD-1.IgV.exon2_RD1_PS3
MGSAPPKKKRKVVDLRTLGYSQQQQEKIKPKVRSTVAQHHEALVGHGFTHAHIVALSQHPAALGTVAVTYQHIITALPEATHEDIVGVGKQWSGARALEALLTDAGELRGPPLQLDTGQLVKIAKRGGVTAMEAVHASRNALTGAPLNLTPDQVVAIASNNGGKQALETVQRLLPVLCQDHGLTPDQVVAIASNGGGKQALETVQRLLPVLCQDHGLTPDQVVAIASHDGGKQALETVQRLLPVLCQDHGLTPDQVVAIASNIGGKQALETVQRLLPVLCQDHGLTPDQVVAIASHDGGKQALETVQRLLPVLCQDHGLTPDQVVAIASNIGGKQALETVQRLLPVLCQDHGLTPDQVVAIASHDGGKQALETVQRLLPVLCQDHGLTPDQVVAIASNIGGKQALETVQRLLPVLCQDHGLTPDQVVAIASNIGGKQALETVQRLLPVLCQDHGLTPDQVVAIASHDGGKQALETVQRLLPVLCQDHGLTPDQVVAIASNGGGKQALETVQRLLPVLCQDHGLTPDQVVAIASNNGGKQALESIVAQLSRPDPALAALTNDHLVALACLGGRPAMDAVKKGLPHAPELIRRVNRRIGERTSHRVAISRVGGSSRRESINPWILTGFADAEGCFLLHIRNLNRTSTKYRTRLSFEIELHNKDKSILENIQSTWKVGIINNIGNRRVRLSVRRFEDLKVIIDHFEKYPLITQKLGDYKLFKQAFSLMENKEHLKENGIKELVRIKAKMNWGLNDELKKAFPENISKERPLINKNIPNLKWLAGFTSGDGNFYVHLKKSGRTTRVYVQLRFSISQHIRDKNLMNSLITYLGCGYITESNPSERSDLEFRVTKFSDINDKIIPVFQENTLIGVKLEDFEDWCKVAKLIEEKKHLTESGLDEIKKIKLNMNKGR

SEQ ID NO: 24 - protein, 236 aa, Mus musculus
MSEPPRAETFVFLDLEATGLPNMDPEIAEISLFAVHRSSLENPERDDSGSLVLPRVLDKLTLCMCPERPFTAKASEITGLSSESLMHCGKAGFNGAVVRTLQGFLSRQEGPICLVAHNGFDYDFPLLCTGLQRLGAHLPQDTVCLDTLPALRGLDRAHSHGTRAQGRKSYSLASLFHRYFQAEPSAAHSAEGDVHTLLLIFLHRAPELLAWADEQARSWAHIEPMYVPPDGPSLEA

SEQ ID NO: 25 - DNA, 22 bp, Homo sapiens
  source 1..22: mol_type = unassigned DNA
aatggtggcatactccgtctgc

SEQ ID NO: 26 - DNA, 11 bp, Homo sapiens
  source 1..11: mol_type = unassigned DNA
tccgctaggaa

SEQ ID NO: 27 - DNA, 37 bp, Homo sapiens
  source 1..37: mol_type = unassigned DNA
tccgctaggaaagacaatggtggcatactccgtctgc

SEQ ID NO: 28 - DNA, 22 bp, Homo sapiens
  source 1..22: mol_type = unassigned DNA
aatggtggcatacaacctttta

SEQ ID NO: 29 - DNA, 22 bp, Homo sapiens
  source 1..22: mol_type = unassigned DNA
tttccacttatactccgtctgc

SEQ ID NO: 30 - DNA, 22 bp, Homo sapiens
  source 1..22: mol_type = unassigned DNA
ggcatgcagatcccacaggcgc

SEQ ID NO: 31 - DNA, 14 bp, Homo sapiens
  source 1..14: mol_type = unassigned DNA
ggtggggctgctcc

SEQ ID NO: 32 - DNA, 37 bp, Homo sapiens
  source 1..37: mol_type = unassigned DNA
ggtggggctgctccaggcatgcagatcccacaggcgc

SEQ ID NO: 33 - DNA, 22 bp, Homo sapiens
  source 1..22: mol_type = unassigned DNA
ggcatgcagatccaacctttta

SEQ ID NO: 34 - DNA, 22 bp, Homo sapiens
  source 1..22: mol_type = unassigned DNA
tttccacttatcccacaggcgc

SEQ ID NO: 35 - DNA, 22 bp, Homo sapiens
  source 1..22: mol_type = unassigned DNA
acgggcgtgacttccacatgag

SEQ ID NO: 36 - DNA, 12 bp, Homo sapiens
  source 1..12: mol_type = unassigned DNA
gtcacacaactg

SEQ ID NO: 37 - DNA, 38 bp, Homo sapiens
  source 1..38: mol_type = unassigned DNA
gtcacacaactgcccaacgggcgtgacttccacatgag

SEQ ID NO: 38 - DNA, 22 bp, Homo sapiens
  source 1..22: mol_type = unassigned DNA
acgggcgtgacttaacctttta

SEQ ID NO: 39 - DNA, 22 bp, Homo sapiens
  source 1..22: mol_type = unassigned DNA
tttccacttacttccacatgag

SEQ ID NO: 40 - RNA, 2650 nt, synthetic construct
  misc_feature 1..2650: note = Synthesized PD-1 Exon5 RD5_CV23MK megaTAL mRNA
  source 1..2650: mol_type = other RNA
atgggatccgccccccccaagaagaagcgcaaggtggtggacctgagaaccctggggtacagccagcagcaacaggagaagatcaaaccgaaggtgcgcagcacggtggcccagcaccatgaagccctcgtgggtcatggattcacgcacgcccacatcgtggccctgtcgcagcatccggccgccctgggcaccgtggcggtgacctaccagcacatcatcaccgccctgcccgaagccacccacgaggacatcgtgggagtgggcaagcagtggtccggagcacgcgccctggaggccctgctgaccgacgccggggaactgcgcggcccgcctctgcagctggataccggccaactggtcaagatcgccaagagaggcggagtgaccgcgatggaggccgtccacgcctcccggaacgctctgaccggtgccccgctcaatctgactccggaccaggtggtggctatcgccagcaacggaggaggaaaacaggccctcgaaacagtgcagaggctgctgcctgtcctttgtcaagatcacgggctgactcccgaccaggtcgtggccattgccagccacgacggcggcaagcaggctttggagactgtgcagcggctcctgccagtgctgtgccaagatcacggtctgaccccagatcaggtcgtcgccattgcttccaacggaggcaaacaagcgctggaaacggtccaacgcctgctgccggtgctttgtcaggatcacggcctgacccctgatcaggtggtggccatcgcgtccaataacggggggaagcaggcactcgagactgtccagaggctcctgcctgtgctctgccaggaccacgggctcacacccgatcaggtcgtcgctatcgcgtcgcacgacggtggaaagcaggccctggaaaccgtgcagcgcctgttgccggtgctgtgtcaggaccatggccttactccggatcaggtcgtcgcgatcgcatctaatggtggaggaaagcaggccctggagacagtccagcgcctgctcccggtgttgtgccaagaccatggtcttacccctgaccaggtggtcgctattgcctcgaacatcggcggaaagcaagccctggaaaccgtgcagcgacttctgccggtcctgtgccaggatcatggattgaccccagaccaggtggtggcgattgccagcaacaacggcgggaagcaagcgttggaaaccgtccagagactgcttcctgtgctgtgccaagaccacggtttgaccccggaccaagtcgtcgccatcgcttccaacaacggagggaagcaggcactcgaaactgtgcaacggttgctgcccgtgctctgtcaggatcacggactcacccctgatcaggtggtggccatcgcaagcaacatcggtggcaaacaggctctggaaactgtccaaagactgctgcccgtgctttgccaggaccacggactgactcctgaccaagtggtggcaattgcctccaacatcggaggcaagcaagcgctcgaatccatcgtggcgcagctcagccggccagaccccgccctggccgccctgactaacgatcacctggtggccctggcgtgcctcggcggtcgccccgctatggacgcggtgaagaaggggctgccccacgcccccgagctcattcggcgggtgaaccgccggatcggagaaagaacctcccatcgggtggccatctcgagatcacggcgggaatccattaacccctggatcctgactggctttgccgacgccgagggatccttccagctcgaaatccggaacgtgaacccaaacatcccccggtatcgcaccagactgcggttcgagatcgaccttcacaacaaggacaagtccattctggaggacatccagtcaacctggaaagtgggaaagatctacaaccagggggactcatacgtgaagctgcgggtgacccgcttcgaagatctcaaagtgatcatcgaccatttcgagaagtaccccctgatcactcagaagcttggagactacaaactgttcaagcaggcattctccgtgatggagaacaaggagcacctgaaggagaacgggattaaggagctggtgcgaattaaggcgaaaatgaactggggattgaacgatgagctgaagaaggcgttcccggaaaacatttccaaggagcgcccgctcatcaacaagaacatccctaatctgaagtggctcgcggggtttacctctggcgacggccatttcggagtgattctcgcaaagcgcaggcccgccagccctgtgcaagtgcggctgcggttcatgatcggccagcacattaaggacaagaacctgatgaactcgctcatcacctaccttggatgcggccggattcgcgaaaagaacaagagcgagaagtcctggctggaatttgaagtgaccaagttcagcgacatcaacgacaagatcattccggtgttccaggaaaacaccctgattggcgtgaagctggaggacttcgaggattggtgcaaggtggccaagctcatcgaagaaaagaagcacctgactgaatccggcttggacgagatcaagaagattaagctgaatatgaacaagggaaggtgatagcgcgctagccgtacggaaaaaaaaaaaaaaaaaa

SEQ ID NO: 41 - RNA, 2526 nt, synthetic construct
  misc_feature 1..2526: note = Synthesized PD-1 Exon1 RD2_B1H8 megaTAL mRNA
  source 1..2526: mol_type = other RNA
atgggaagcgccccgccgaagaagaagcgcaaggtggtggatctgagaaccctgggatacagccagcagcagcaggagaagatcaagccgaaggtccggtctaccgtggcccagcaccatgaggcccttgtgggccacggcttcacacatgcacacatcgtcgccctgtcgcagcatcccgccgccctggggaccgtggccgtgacctatcaacacatcattaccgccctgccggaggccacccacgaggacatcgtgggtgtggggaagcagtggagcggagccagggcactcgaagccctcctcactgacgctggagaactgcgcggaccgcctctccagctggacaccggacagctggtgaaaatcgccaagcggggaggagtgaccgccatggaagccgtgcacgcctcgaggaacgcgctgactggcgcccctctgaacctgacccctgatcaggtcgtggctatcgcctcaaacaacgggggtaagcaggcgctggagacagtgcaacgacttctgccagtgctttgtcaggaccatggtctgacccccgaccaggtcgtcgccattgcatccaacaatggtggcaagcaggcactggagactgtccagaggctgctcccggtgctgtgccaggaccacgggctcaccccggaccaagtggtcgccatcgcctccaacggaggaggaaaacaagctctggagactgtgcaacgcctgctgcctgtgttgtgccaagaccacggactgacgcccgatcaggtggtggcgatcgcatcgaacaacggaggaaagcaagcgctggaaaccgtgcagcgcctcctgcccgtcctctgccaggatcacggcctgactccggaccaggtggtcgcgatcgccagcaataacggggggaagcaagccctcgagactgtgcagcggttgctgcccgtgctctgccaagatcatggccttaccccagaccaagtcgtggccattgcttccaacaacggtggcaaacaggcgctcgaaaccgtccagcggctgttgcccgtgctttgccaggatcacggactcacccctgatcaggtggtggcaattgcgtccaacaacggtggaaagcaggccctggaaacggtgcagcggctgcttccggtcctgtgtcaggatcatgggctgactcccgaccaggtcgtcgccattgcatcccacgatgggggtaaacaggccctcgaaacagtgcagagactcctgccagtcctgtgccaagaccacggacttaccccggatcaggtggtggccatagcctcgaacggcggcgggaaacaggctctggaaactgtgcaaagactcctcccggtgttgtgtcaagaccatggactgaccccagatcaggtggtggctattgcctctaacaacggcggcaagcaagcactcgaaagcatcgtggcccagttgtcacgccccgaccccgcactggctgccctgacgaatgaccatctggtggcgctggcctgcctgggagggaggccagcgatggatgcggtgaagaagggactgccccatgctccggagctgattcggagagtgaataggcgcatcggagagagaacttcacatcgggtggccatttctagagtgggcggcagctcccggcgcgagtccattaacccctggatcctgaccggctttgccgacgccgaagggtccttcggcctctcgatcctgaaccggaaccggggtaccgctcggtaccacaccagactgtccttcaccatcgtgctgcacaacaaggacaagagcatcctcgaaaacattcagtcaacgtggaaggtgggaattattactaacgacggcgacagatacgtgcgcctgtgcgtgacccggtttgaggacctgaaggtcattatcgaccacttcgagaagtaccccctcgtgactcagaagctgggagactacaagctgttcaagcaggcgttctcggtgatggaaaacaaggagcacctgaaggagaacggcatcaaggagctcgcccggatcaaggccaagatgaactggggcctgaatgatgaactcaagaaggcgttccctgaaaacatcggtaaagaacggcccctgatcaacaagaacatcccgaacttcaagtggcttgccggattcacctccggcgacggatccttcttcgtccggctgcgcaagtccaacgtgaacgcgagagtgcgggtgcaattggtctttgaaatctcacagcacatcagggacaagaatttgatgaactccctcatcacctacctgggttgcggacacatctacgaaggcaataagtcggagcggagctggctgcagtttcgcgtggaaaagttctccgacattaacgacaagatcatcccagtgttccaggaaaacactctgattggcgtgaagcttgaggatttcgaggactggtgcaaggtggccaagctgattgaagagaagaagcacctgaccgagtccggcctggacgaaatcaagaaaatcaagctgaacatgaacaagggacggtga

SEQ ID NO: 42 - RNA, 2730 nt, synthetic construct
  misc_feature 1..2730: note = Synthesized PD-1 Exon2 RD1_G5 megaTAL mRNA
  source 1..2730: mol_type = other RNA
atgggaagcgcccctccgaagaagaagcgcaaggtcgtggacctcagaaccctgggttactcccagcagcagcaggagaaaattaagccgaaggtgcgctccaccgtggctcaacaccacgaggccctcgtgggccatggattcactcacgcccatatcgtggccctgtcccagcacccggccgccctgggcaccgtggcggtgacctaccagcacatcatcaccgcgctgcctgaagccacccacgaggacatcgtcggtgtgggtaagcagtggtccggagccagagccctggaggctctgctgaccgacgccggagaactcagaggcccgcctctgcagctggacaccggacagctggtgaagatagccaagagaggcggcgtgaccgccatggaagccgtgcatgcgtcccgcaacgcactgaccggggcccccctgaacctgactccagaccaagtggtggctatcgccagcaacaatggaggaaagcaagccttggaaaccgtgcagcggctgctcccggtcctttgccaagaccacggcctgacacccgatcaggtggtggcaatcgcatcgaatggcggcgggaagcaggccctcgagactgtgcagaggctcctgcctgtgctgtgccaggaccatgggctgaccccagaccaggtggtcgcaatcgcctcgcacgacggaggcaagcaagccctggaaactgtccagcgcctgctccctgtcctgtgtcaagatcatgggctcactcctgatcaggtcgtcgccatcgcctcgaacattggtggcaagcaggcgctcgaaaccgtccagcggttgctgccagtgctttgccaggaccatggtctgacccccgatcaagtggtcgcgattgcctcacacgatggcggtaagcaggctttggaaaccgtgcaacggctgttgcctgtcctctgccaggaccacggcttgactcccgaccaggtggtggccatagcctcaaacatcggagggaaacaagccctcgaaaccgtccagaggctgctgccggtgttgtgccaggatcacggattgaccccagaccaggtggtcgccattgcttcccacgatgggggaaagcaggccctggagactgtgcagcgcctccttcccgtcctgtgtcaggatcatggacttacccccgaccaagtcgtggcgattgcttccaatatcggaggcaaacaggcccttgaaacagtgcagcgcctgttgccggtgctctgccaagatcacggactgacccctgaccaggtggtggcgatcgcgtcaaatatcggcggcaagcaggcactggagacagtccagagactcctgccggtcctctgccaggaccacggtcttactcctgaccaagtggtggctatcgcatcccatgatggtgggaaacaggctcttgaaactgtgcaacgcctgctgcccgtgctgtgccaagaccacggactgactccggaccaggtcgtggccatcgcttcaaacggagggggaaaacaggcacttgaaacggtgcagagactgctgcctgtcctttgtcaggaccacgggttgaccccggaccaggtcgtggctattgcctcgaacaacggggggaagcaagcgctcgagtccattgtggcccagctgagccggcctgatcccgcactggccgcgctgaccaacgatcacctggtggccctcgcctgtctgggcggacggccggccatggacgccgtgaagaagggactgccgcacgcgcccgagctgatccgccgcgtgaacaggcggattggagaacgcacctcccaccgggtggccatctcgagagtgggaggatcctctagacgggagtccattaacccgtggatcctgactggattcgccgacgccgaggggtccttccagctgtacatctccaacgtgaacaacaaccgcagcagatacagggcccggctgcggttcgcgatcgaactgcacaataaggacaagagcatcctcgagaacattcagtccacttggaaggtgggcgtgattaacaacatcggcgataccagcgtgcggctctccgtggggcggttcgaagatctcaaggtgatcatcgaccacttcgagaagtacccgctgatcacccagaagctgggagactacaagctgttcaagcaagctttcagcgtgatggaaaacaaggaacatctgaaagagaacggtatcaaggaactggtgcggattaaggccaagatgaactggggtctgaacgatgaactgaagaaggcgttcccggagaatatcagcaaggagcgccccctgattaacaaaaacatcccaaacctcaagtggctcgccggctttacttccggagatggtaacttctacgtgcacctgaagaagtccggaagaaccacccgggtctacgtgcagctgaggttctccatcgcccagcacatccgggacaagaacttgatgaactccctgatcacctacctcggttgcggatacatcaacgaatggaacgccagcgagagatcggccctggagttcagggtgactaagttctccgacatcaacgacaagattatccccgtgtttcaggaaaataccctcatcggcgtgaagctggaggactttgaggactggtgcaaggtggccaagctgatcgaggaaaagaaacatctgaccgagagcggcctggacgaaatcaagaagattaagctgaacatgaacaagggacgatga

SEQ ID NO: 43 - RNA, 711 nt, Mus musculus
  source 1..711: mol_type = unassigned RNA
atgtctgagccacctcgggctgagacctttgtattcctggacctagaagccactgggctcccaaacatggaccctgagattgcagagatatccctttttgctgttcaccgctcttccctggagaacccagaacgggatgattctggttccttggtgctgccccgtgttctggacaagctcacactgtgcatgtgcccggagcgcccctttactgccaaggccagtgagattactggtttgagcagcgaaagcctgatgcactgcgggaaggctggtttcaatggcgctgtggtaaggacactgcagggcttcctaagccgccaggagggccccatctgccttgtggcccacaatggcttcgattatgacttcccactgctgtgcacggggctacaacgtctgggtgcccatctgccccaagacactgtctgcctggacacactgcctgcattgcggggcctggaccgtgctcacagccacggcaccagggctcaaggccgcaaaagctacagcctggccagtctcttccaccgctacttccaggctgaacccagtgctgcccattcagcagaaggtgatgtgcacaccctgcttctgatcttcctgcatcgtgctcctgagctgctcgcctgggcagatgagcaggcccgcagctgggctcatattgagcccatgtacgtgccacctgatggtccaagcctcgaagcctga

SEQ ID NO: 44 - DNA, 7601 bp, synthetic construct
  misc_feature 1..7601: note = Synthesized rAAV PD-1 Exon5_MND-BFP construct
  source 1..7601: mol_type = other DNA
cagctgcgcgctcgctcgctcactgaggccgcccgggcaaagcccgggcgtcgggcgacctttggtcgcccggcctcagtgagcgagcgagcgcgcagagagggagtggccaactccatcactaggggttccttgtagttaatgattaacccgccatgctacttatctacgtagaattcagtccagggctctgtcctgcacctggggaatggtgaccggcatctctgtcctctagctctggaagcaccccagcccctctagtctgccctcacccctgaccctgaccctccaccctgaccccgtcctaacccctgacctttgtgcccttccagagagaagggcagaagtgcccacagcccaccccagcccctcacccaggccagccggccagttccaaaccctggtggttggtgtcgtgggcggcctgctgggcagcctggtgctgctagtctgggtcctggccgtcatctgctcccgggccgcacgaggtaacgtcatcccagcccctcggcctgccctgccctaaccctgctggcggccctcactcccgcctccccttcctccacccttccctcaccccaccccacctccccccatctccccgccaggctaagtccctgatgaaggcccctggactaagaccccccacctaggagcacggctcagggtcggcctggtgaccccaagtgtgtttctctgcagggacaataggagccaggcgcaccggccagcccctggtgagtctcactcttttcctgcatgatccactgtgccttccttcctgggtgggcagaggtggaaggacaggctgggaccacacggcctgcaggactcacattctattatagccaggaccccacctccccagcccccaggcagcaacctcaatccctaaagccatgatctggggccccagcccacctgcggtctccgggggtgcccggcccatgtgtgtgcctgcctgcggtctccaggggtgcctggcccacgcgtgtgcccgcctgcggtctctgggggtgcccggcccacatatgtgcctgcctgcggtctccaggtgtgcccggcccatgcgtgtgcccacctgcgagggcgtggggtgggcttggtcatttcttatcttacattggagacaggagagcttgaaaagtcacattttggaatcctaaatctgcaagaatgccagggacatttcagagggggacattgagccagagaggaggggtggtgtccccagatcacacagagggcagtggtgggacagctcagggtaagcagctcatagtggggggcccaggttcggtgccggtactgcagccaggctgtggagccgcgggcctccttcctgcggtgggccgtggggctgactccctctccctttctcctcaaagaaggaggacccctcagccgtgcctgtgttctctgtggactatggggagctggatttccagtggcgagagaagaccccggagccccccgtgccctgtgtccctgagcagacggagtaatgcatgaacagagaaacaggagaatatgggccaaacaggatatctgtggtaagcagttcctgccccggctcagggccaagaacagttggaacagcagaatatgggccaaacaggatatctgtggtaagcagttcctgccccggctcagggccaagaacagatggtccccagatgcggtcccgccctcagcagtttctagagaaccatcagatgtttccagggtgccccaaggacctgaaatgaccctgtgccttatttgaactaaccaatcagttcgcttctcgcttctgttcgcgcgcttctgctccccgagctctatataagcagagctcgtttagtgaaccgtcagatcgcctggagacgccatccacgctgttttgacttccatagaaggatctcgaggccaccatggctagcgagctgattaaggagaacatgcacatgaagctgtacatggagggcaccgtggacaaccatcacttcaagtgcacatccgagggcgaaggcaagccctacgagggcacccagaccatgagaatcaaggtggtcgagggcggccctctccccttcgccttcgacatcctggctactagcttcctctacggcagcaagaccttcatcaaccacacccagggcatccccgacttcttcaagcagtccttccctgagggcttcacatgggagagagtcaccacatacgaggacgggggcgtgctgaccgctacccaggacaccagcctccaggacggctgcctcatctacaacgtcaagatcagaggggtgaacttcacatccaacggccctgtgatgcagaagaaaacactcggctgggaggccttcaccgagacgctgtaccccgctgacggcggcctggaaggcagaaacgacatggccctgaagctcgtgggcgggagccatctgatcgcaaacatcaagaccacatatagatccaagaaacccgctaagaacctcaagatgcctggcgtctactatgtggactacagactggaaagaatcaaggaggccaacaacgagacctacgtcgagcagcacgaggtggcagtggccagatactgcgacctccctagcaaactggggcacaagctaaattgaaagctttgctttatttgtgaaatttgtgatgctattgctttatttgtaaccattataagctgcaataaacaagtttaacaacaacaattgcattcattttatgtttcaggttcagggggaggtgtgggaggttttttaaagtcgacccaccattgtctttcctagcggaatgggcacctcatcccccgcccgcaggggctcagctgacggccctcggagtgcccagccactgaggcctgaggatggacactgctcttggcccctctgaccggcttccttggccaccagtgttctgcagaccctccaccatgagcccgggtcagcgcatttcctcaggagaagcaggcagggtgcaggccattgcaggccgtccaggggctgagctgcctgggggcgaccggggctccagcctgcacctgcaccaggcacagccccaccacaggactcatgtctcaatgcccacagtgagcccaggcagcaggtgtcaccgtcccctacagggagggccagatgcagtcactgcttcaggtcctgccagcacagagctgcctgcgtccagctccctgaatctctgctgctgctgctgctgctgctgctgctgcctgcggcccggggctgaaggcgccgtggccctgcctgacgccccggagcctcctgcctgaacttgggggctggttggagatggccttggagcagccaaggtgcccctggcagtggcatcccgaaacgccctggacgcagggcccaagactgggcacaggagtgggaggtacatggggctggggactccccaggagttatctgctccctgcaggcctagagaagtttcagggaaggtcagaagagctcctggctgtggtgggcagggcaggaaacccctccacctttacacatgcccaggcagcacctcaggccctttgtggggcagggaagctgaggcagtaagcgggcaggcagagctggaggcctttcaggcccagccagcactctggcctcctgccgccgcattccaccccagcccctcacaccactcgggagagggacatcctacggtcccaaggtcaggagggcagggctggggttgactcaggcccctcccagctgtggccacctgggtgttgggagggcagaagtgcaggcacctagggccccccatgtgcccaccctgggagctctccttggaacccattcctgaaattatttaaaggggttggccggactagttacgtagataagtagcatggcgggttaatcattaactacaaggaacccctagtgatggagttggccactccctctctgcgcgctcgctcgctcactgaggccgggcgaccaaaggtcgcccgacgcccgggctttgcccgggcggcctcagtgagcgagcgagcgcgccagctggcgtaatagcgaagaggcccgcaccgatcgcccttcccaacagttgcgcagcctgaatggcgaatggcgattccgttgcaatggctggcggtaatattgttctggatattaccagcaaggccgatagtttgagttcttctactcaggcaagtgatgttattactaatcaaagaagtattgcgacaacggttaatttgcgtgatggacagactcttttactcggtggcctcactgattataaaaacacttctcaggattctggcgtaccgttcctgtctaaaatccctttaatcggcctcctgtttagctcccgctctgattctaacgaggaaagcacgttatacgtgctcgtcaaagcaaccatagtacgcgccctgtagcggcgcattaagcgcggcgggtgtggtggttacgcgcagcgtgaccgctacacttgccagcgccctagcgcccgctcctttcgctttcttcccttcctttctcgccacgttcgccggctttccccgtcaagctctaaatcgggggctccctttagggttccgatttagtgctttacggcacctcgaccccaaaaaacttgattagggtgatggttcacgtagtgggccatcgccctgatagacggtttttcgccctttgacgttggagtccacgttctttaatagtggactcttgttccaaactggaacaacactcaaccctatctcggtctattcttttgatttataagggattttgccgatttcggcctattggttaaaaaatgagctgatttaacaaaaatttaacgcgaattttaacaaaatattaacgtttacaatttaaatatttgcttatacaatcttcctgtttttggggcttttctgattatcaaccggggtacatatgattgacatgctagttttacgattaccgttcatcgattctcttgtttgctccagactctcaggcaatgacctgatagcctttgtagagacctctcaaaaatagctaccctctccggcatgaatttatcagctagaacggttgaatatcatattgatggtgatttgactgtctccggcctttctcacccgtttgaatctttacctacacattactcaggcattgcatttaaaatatatgagggttctaaaaatttttatccttgcgttgaaataaaggcttctcccgcaaaagtattacagggtcataatgtttttggtacaaccgatttagctttatgctctgaggctttattgcttaattttgctaattctttgccttgcctgtatgatttattggatgttggaatcgcctgatgcggtattttctccttacgcatctgtgcggtatttcacaccgcatatggtgcactctcagtacaatctgctctgatgccgcatagttaagccagccccgacacccgccaacacccgctgacgcgccctgacgggcttgtctgctcccggcatccgcttacagacaagctgtgaccgtctccgggagctgcatgtgtcagaggttttcaccgtcatcaccgaaacgcgcgagacgaaagggcctcgtgatacgcctatttttataggttaatgtcatgataataatggtttcttagacgtcaggtggcacttttcggggaaatgtgcgcggaacccctatttgtttatttttctaaatacattcaaatatgtatccgctcatgagacaataaccctgataaatgcttcaataatattgaaaaaggaagagtatgagtattcaacatttccgtgtcgcccttattcccttttttgcggcattttgccttcctgtttttgctcacccagaaacgctggtgaaagtaaaagatgctgaagatcagttgggtgcacgagtgggttacatcgaactggatctcaacagcggtaagatccttgagagttttcgccccgaagaacgttttccaatgatgagcacttttaaagttctgctatgtggcgcggtattatcccgtattgacgccgggcaagagcaactcggtcgccgcatacactattctcagaatgacttggttgagtactcaccagtcacagaaaagcatcttacggatggcatgacagtaagagaattatgcagtgctgccataaccatgagtgataacactgcggccaacttacttctgacaacgatcggaggaccgaaggagctaaccgcttttttgcacaacatgggggatcatgtaactcgccttgatcgttgggaaccggagctgaatgaagccataccaaacgacgagcgtgacaccacgatgcctgtagcaatggcaacaacgttgcgcaaactattaactggcgaactacttactctagcttcccggcaacaattaatagactggatggaggcggataaagttgcaggaccacttctgcgctcggcccttccggctggctggtttattgctgataaatctggagccggtgagcgtgggtctcgcggtatcattgcagcactggggccagatggtaagccctcccgtatcgtagttatctacacgacggggagtcaggcaactatggatgaacgaaatagacagatcgctgagataggtgcctcactgattaagcattggtaactgtcagaccaagtttactcatatatactttagattgatttaaaacttcatttttaatttaaaaggatctaggtgaagatcctttttgataatctcatgaccaaaatcccttaacgtgagttttcgttccactgagcgtcagaccccgtagaaaagatcaaaggatcttcttgagatcctttttttctgcgcgtaatctgctgcttgcaaacaaaaaaaccaccgctaccagcggtggtttgtttgccggatcaagagctaccaactctttttccgaaggtaactggcttcagcagagcgcagataccaaatactgtccttctagtgtagccgtagttaggccaccacttcaagaactctgtagcaccgcctacatacctcgctctgctaatcctgttaccagtggctgctgccagtggcgataagtcgtgtcttaccgggttggactcaagacgatagttaccggataaggcgcagcggtcgggctgaacggggggttcgtgcacacagcccagcttggagcgaacgacctacaccgaactgagatacctacagcgtgagctatgagaaagcgccacgcttcccgaagggagaaaggcggacaggtatccggtaagcggcagggtcggaacaggagagcgcacgagggagcttccagggggaaacgcctggtatctttatagtcctgtcgggtttcgccacctctgacttgagcgtcgatttttgtgatgctcgtcaggggggcggagcctatggaaaaacgccagcaacgcggcctttttacggttcctggccttttgctggccttttgctcacatgttctttcctgcgttatcccctgattctgtggataaccgtattaccgcctttgagtgagctgataccgctcgccgcagccgaacgaccgagcgcagcgagtcagtgagcgaggaagcggaagagcgcccaatacgcaaaccgcctctccccgcgcgttggccgattcattaatg

SEQ ID NO: 45 - DNA, 1325 bp, Homo sapiens
  source 1..1325: mol_type = unassigned DNA
agtccagggctctgtcctgcacctggggaatggtgaccggcatctctgtcctctagctctggaagcaccccagcccctctagtctgccctcacccctgaccctgaccctccaccctgaccccgtcctaacccctgacctttgtgcccttccagagagaagggcagaagtgcccacagcccaccccagcccctcacccaggccagccggccagttccaaaccctggtggttggtgtcgtgggcggcctgctgggcagcctggtgctgctagtctgggtcctggccgtcatctgctcccgggccgcacgaggtaacgtcatcccagcccctcggcctgccctgccctaaccctgctggcggccctcactcccgcctccccttcctccacccttccctcaccccaccccacctccccccatctccccgccaggctaagtccctgatgaaggcccctggactaagaccccccacctaggagcacggctcagggtcggcctggtgaccccaagtgtgtttctctgcagggacaataggagccaggcgcaccggccagcccctggtgagtctcactcttttcctgcatgatccactgtgccttccttcctgggtgggcagaggtggaaggacaggctgggaccacacggcctgcaggactcacattctattatagccaggaccccacctccccagcccccaggcagcaacctcaatccctaaagccatgatctggggccccagcccacctgcggtctccgggggtgcccggcccatgtgtgtgcctgcctgcggtctccaggggtgcctggcccacgcgtgtgcccgcctgcggtctctgggggtgcccggcccacatatgtgcctgcctgcggtctccaggtgtgcccggcccatgcgtgtgcccacctgcgagggcgtggggtgggcttggtcatttcttatcttacattggagacaggagagcttgaaaagtcacattttggaatcctaaatctgcaagaatgccagggacatttcagagggggacattgagccagagaggaggggtggtgtccccagatcacacagagggcagtggtgggacagctcagggtaagcagctcatagtggggggcccaggttcggtgccggtactgcagccaggctgtggagccgcgggcctccttcctgcggtgggccgtggggctgactccctctccctttctcctcaaagaaggaggacccctcagccgtgcctgtgttctctgtggactatggggagctggatttccagtggcgagagaagaccccggagccccccgtgccctgtgtccctgagcagacggagta

SEQ ID NO: 46 - DNA, 1072 bp, Homo sapiens
  source 1..1072: mol_type = unassigned DNA
ccaccattgtctttcctagcggaatgggcacctcatcccccgcccgcaggggctcagctgacggccctcggagtgcccagccactgaggcctgaggatggacactgctcttggcccctctgaccggcttccttggccaccagtgttctgcagaccctccaccatgagcccgggtcagcgcatttcctcaggagaagcaggcagggtgcaggccattgcaggccgtccaggggctgagctgcctgggggcgaccggggctccagcctgcacctgcaccaggcacagccccaccacaggactcatgtctcaatgcccacagtgagcccaggcagcaggtgtcaccgtcccctacagggagggccagatgcagtcactgcttcaggtcctgccagcacagagctgcctgcgtccagctccctgaatctctgctgctgctgctgctgctgctgctgctgcctgcggcccggggctgaaggcgccgtggccctgcctgacgccccggagcctcctgcctgaacttgggggctggttggagatggccttggagcagccaaggtgcccctggcagtggcatcccgaaacgccctggacgcagggcccaagactgggcacaggagtgggaggtacatggggctggggactccccaggagttatctgctccctgcaggcctagagaagtttcagggaaggtcagaagagctcctggctgtggtgggcagggcaggaaacccctccacctttacacatgcccaggcagcacctcaggccctttgtggggcagggaagctgaggcagtaagcgggcaggcagagctggaggcctttcaggcccagccagcactctggcctcctgccgccgcattccaccccagcccctcacaccactcgggagagggacatcctacggtcccaaggtcaggagggcagggctggggttgactcaggcccctcccagctgtggccacctgggtgttgggagggcagaagtgcaggcacctagggccccccatgtgcccaccctgggagctctccttggaacccattcctgaaattatttaaaggggttggccgg

SEQ ID NO: 47 - DNA, 7601 bp, synthetic construct
  misc_feature 1..7601: note = Synthesized rAAV PD-1 Exon5_MND-BFP 3'-Homology Arm SNP construct
  source 1..7601: mol_type = other DNA
cagctgcgcgctcgctcgctcactgaggccgcccgggcaaagcccgggcgtcgggcgacctttggtcgcccggcctcagtgagcgagcgagcgcgcagagagggagtggccaactccatcactaggggttccttgtagttaatgattaacccgccatgctacttatctacgtagaattcagtccagggctctgtcctgcacctggggaatggtgaccggcatctctgtcctctagctctggaagcaccccagcccctctagtctgccctcacccctgaccctgaccctccaccctgaccccgtcctaacccctgacctttgtgcccttccagagagaagggcagaagtgcccacagcccaccccagcccctcacccaggccagccggccagttccaaaccctggtggttggtgtcgtgggcggcctgctgggcagcctggtgctgctagtctgggtcctggccgtcatctgctcccgggccgcacgaggtaacgtcatcccagcccctcggcctgccctgccctaaccctgctggcggccctcactcccgcctccccttcctccacccttccctcaccccaccccacctccccccatctccccgccaggctaagtccctgatgaaggcccctggactaagaccccccacctaggagcacggctcagggtcggcctggtgaccccaagtgtgtttctctgcagggacaataggagccaggcgcaccggccagcccctggtgagtctcactcttttcctgcatgatccactgtgccttccttcctgggtgggcagaggtggaaggacaggctgggaccacacggcctgcaggactcacattctattatagccaggaccccacctccccagcccccaggcagcaacctcaatccctaaagccatgatctggggccccagcccacctgcggtctccgggggtgcccggcccatgtgtgtgcctgcctgcggtctccaggggtgcctggcccacgcgtgtgcccgcctgcggtctctgggggtgcccggcccacatatgtgcctgcctgcggtctccaggtgtgcccggcccatgcgtgtgcccacctgcgagggcgtggggtgggcttggtcatttcttatcttacattggagacaggagagcttgaaaagtcacattttggaatcctaaatctgcaagaatgccagggacatttcagagggggacattgagccagagaggaggggtggtgtccccagatcacacagagggcagtggtgggacagctcagggtaagcagctcatagtggggggcccaggttcggtgccggtactgcagccaggctgtggagccgcgggcctccttcctgcggtgggccgtggggctgactccctctccctttctcctcaaagaaggaggacccctcagccgtgcctgtgttctctgtggactatggggagctggatttccagtggcgagagaagaccccggagccccccgtgccctgtgtccctgagcagacggagtaatgcatgaacagagaaacaggagaatatgggccaaacaggatatctgtggtaagcagttcctgccccggctcagggccaagaacagttggaacagcagaatatgggccaaacaggatatctgtggtaagcagttcctgccccggctcagggccaagaacagatggtccccagatgcggtcccgccctcagcagtttctagagaaccatcagatgtttccagggtgccccaaggacctgaaatgaccctgtgccttatttgaactaaccaatcagttcgcttctcgcttctgttcgcgcgcttctgctccccgagctctatataagcagagctcgtttagtgaaccgtcagatcgcctggagacgccatccacgctgttttgacttccatagaaggatctcgaggccaccatggctagcgagctgattaaggagaacatgcacatgaagctgtacatggagggcaccgtggacaaccatcacttcaagtgcacatccgagggcgaaggcaagccctacgagggcacccagaccatgagaatcaaggtggtcgagggcggccctctccccttcgccttcgacatcctggctactagcttcctctacggcagcaagaccttcatcaaccacacccagggcatccccgacttcttcaagcagtccttccctgagggcttcacatgggagagagtcaccacatacgaggacgggggcgtgctgaccgctacccaggacaccagcctccaggacggctgcctcatctacaacgtcaagatcagaggggtgaacttcacatccaacggccctgtgatgcagaagaaaacactcggctgggaggccttcaccgagacgctgtaccccgctgacggcggcctggaaggcagaaacgacatggccctgaagctcgtgggcgggagccatctgatcgcaaacatcaagaccacatatagatccaagaaacccgctaagaacctcaagatgcctggcgtctactatgtggactacagactggaaagaatcaaggaggccaacaacgagacctacgtcgagcagcacgaggtggcagtggccagatactgcgacctccctagcaaactggggcacaagctaaattgaaagctttgctttatttgtgaaatttgtgatgctattgctttatttgtaaccattataagctgcaataaacaagtttaacaacaacaattgcattcattttatgtttcaggttcagggggaggtgtgggaggttttttaaagtcgacccaccattgtctttcctagcggaatgggcacctcatcccccgcccgcaggggctcagccgacggccctcggagtgcccagccactgaggcctgaggatggacactgctcttggcccctctgaccggcttccttggccaccagtgttctgcagaccctccaccatgagcccgggtcagcgcatttcctcaggagaagcaggcagggtgcaggccattgcaggccgtccaggggctgagctgcctgggggcgaccggggctccagcctgcacctgcaccaggcacagccccaccacaggactcatgtctcaatgcccacagtgagcccaggcagcaggtgtcaccgtcccctacagggagggccagatgcagtcactgcttcaggtcctgccagcacagagctgcctgcgtccagctccctgaatctctgctgctgctgctgctgctgctgctgctgcctgcggcccggggctgaaggcgccgtggccctgcctgacgccccggagcctcctgcctgaacttgggggctggttggagatggccttggagcagccaaggtgcccctggcagtggcatcccgaaacgccctggacgcagggcccaagactgggcacaggagtgggaggtacatggggctggggactccccaggagttatctgctccctgcaggcctagagaagtttcagggaaggtcagaagagctcctggctgtggtgggcagggcaggaaacccctccacctttacacatgcccaggcagcacctcaggccctttgtggggcagggaagctgaggcagtaagcgggcaggcagagctggaggcctttcaggcccagccagcactctggcctcctgccgccgcattccaccccagcccctcacaccactcgggagagggacatcctacggtcccaaggtcaggagggcagggctggggttgactcaggcccctcccagctgtggccacctgggtgttgggagggcagaagtgcaggcacctagggccccccatgtgcccaccctgggagctctccttggaacccattcctgaaattatttaaaggggttggccggactagttacgtagataagtagcatggcgggttaatcattaactacaaggaacccctagtgatggagttggccactccctctctgcgcgctcgctcgctcactgaggccgggcgaccaaaggtcgcccgacgcccgggctttgcccgggcggcctcagtgagcgagcgagcgcgccagctggcgtaatagcgaagaggcccgcaccgatcgcccttcccaacagttgcgcagcctgaatggcgaatggcgattccgttgcaatggctggcggtaatattgttctggatattaccagcaaggccgatagtttgagttcttctactcaggcaagtgatgttattactaatcaaagaagtattgcgacaacggttaatttgcgtgatggacagactcttttactcggtggcctcactgattataaaaacacttctcaggattctggcgtaccgttcctgtctaaaatccctttaatcggcctcctgtttagctcccgctctgattctaacgaggaaagcacgttatacgtgctcgtcaaagcaaccatagtacgcgccctgtagcggcgcattaagcgcggcgggtgtggtggttacgcgcagcgtgaccgctacacttgccagcgccctagcgcccgctcctttcgctttcttcccttcctttctcgccacgttcgccggctttccccgtcaagctctaaatcgggggctccctttagggttccgatttagtgctttacggcacctcgaccccaaaaaacttgattagggtgatggttcacgtagtgggccatcgccctgatagacggtttttcgccctttgacgttggagtccacgttctttaatagtggactcttgttccaaactggaacaacactcaaccctatctcggtctattcttttgatttataagggattttgccgatttcggcctattggttaaaaaatgagctgatttaacaaaaatttaacgcgaattttaacaaaatattaacgtttacaatttaaatatttgcttatacaatcttcctgtttttggggcttttctgattatcaaccggggtacatatgattgacatgctagttttacgattaccgttcatcgattctcttgtttgctccagactctcaggcaatgacctgatagcctttgtagagacctctcaaaaatagctaccctctccggcatgaatttatcagctagaacggttgaatatcatattgatggtgatttgactgtctccggcctttctcacccgtttgaatctttacctacacattactcaggcattgcatttaaaatatatgagggttctaaaaatttttatccttgcgttgaaataaaggcttctcccgcaaaagtattacagggtcataatgtttttggtacaaccgatttagctttatgctctgaggctttattgcttaattttgctaattctttgccttgcctgtatgatttattggatgttggaatcgcctgatgcggtattttctccttacgcatctgtgcggtatttcacaccgcatatggtgcactctcagtacaatctgctctgatgccgcatagttaagccagccccgacacccgccaacacccgctgacgcgccctgacgggcttgtctgctcccggcatccgcttacagacaagctgtgaccgtctccgggagctgcatgtgtcagaggttttcaccgtcatcaccgaaacgcgcgagacgaaagggcctcgtgatacgcctatttttataggttaatgtcatgataataatggtttcttagacgtcaggtggcacttttcggggaaatgtgcgcggaacccctatttgtttatttttctaaatacattcaaatatgtatccgctcatgagacaataaccctgataaatgcttcaataatattgaaaaaggaagagtatgagtattcaacatttccgtgtcgcccttattcccttttttgcggcattttgccttcctgtttttgctcacccagaaacgctggtgaaagtaaaagatgctgaagatcagttgggtgcacgagtgggttacatcgaactggatctcaacagcggtaagatccttgagagttttcgccccgaagaacgttttccaatgatgagcacttttaaagttctgctatgtggcgcggtattatcccgtattgacgccgggcaagagcaactcggtcgccgcatacactattctcagaatgacttggttgagtactcaccagtcacagaaaagcatcttacggatggcatgacagtaagagaattatgcagtgctgccataaccatgagtgataacactgcggccaacttacttctgacaacgatcggaggaccgaaggagctaaccgcttttttgcacaacatgggggatcatgtaactcgccttgatcgttgggaaccggagctgaatgaagccataccaaacgacgagcgtgacaccacgatgcctgtagcaatggcaacaacgttgcgcaaactattaactggcgaactacttactctagcttcccggcaacaattaatagactggatggaggcggataaagttgcaggaccacttctgcgctcggcccttccggctggctggtttattgctgataaatctggagccggtgagcgtgggtctcgcggtatcattgcagcactggggccagatggtaagccctcccgtatcgtagttatctacacgacggggagtcaggcaactatggatgaacgaaatagacagatcgctgagataggtgcctcactgattaagcattggtaactgtcagaccaagtttactcatatatactttagattgatttaaaacttcatttttaatttaaaaggatctaggtgaagatcctttttgataatctcatgaccaaaatcccttaacgtgagttttcgttccactgagcgtcagaccccgtagaaaagatcaaaggatcttcttgagatcctttttttctgcgcgtaatctgctgcttgcaaacaaaaaaaccaccgctaccagcggtggtttgtttgccggatcaagagctaccaactctttttccgaaggtaactggcttcagcagagcgcagataccaaatactgtccttctagtgtagccgtagttaggccaccacttcaagaactctgtagcaccgcctacatacctcgctctgctaatcctgttaccagtggctgctgccagtggcgataagtcgtgtcttaccgggttggactcaagacgatagttaccggataaggcgcagcggtcgggctgaacggggggttcgtgcacacagcccagcttggagcgaacgacctacaccgaactgagatacctacagcgtgagctatgagaaagcgccacgcttcccgaagggagaaaggcggacaggtatccggtaagcggcagggtcggaacaggagagcgcacgagggagcttccagggggaaacgcctggtatctttatagtcctgtcgggtttcgccacctctgacttgagcgtcgatttttgtgatgctcgtcaggggggcggagcctatggaaaaacgccagcaacgcggcctttttacggttcctggccttttgctggccttttgctcacatgttctttcctgcgttatcccctgattctgtggataaccgtattaccgcctttgagtgagctgataccgctcgccgcagccgaacgaccgagcgcagcgagtcagtgagcgaggaagcggaagagcgcccaatacgcaaaccgcctctccccgcgcgttggccgattcattaatg

SEQ ID NO: 48 - DNA, 7601 bp, synthetic construct
  misc_feature 1..7601: note = Synthesized rAAV PD-1 Exon5_MND-BFP 5'-Homology Arm SNP construct
  source 1..7601: mol_type = other DNA
cagctgcgcgctcgctcgctcactgaggccgcccgggcaaagcccgggcgtcgggcgacctttggtcgcccggcctcagtgagcgagcgagcgcgcagagagggagtggccaactccatcactaggggttccttgtagttaatgattaacccgccatgctacttatctacgtagaattcagtccagggctctgtcctgcacctggggaatggtgaccggcatctctgtcctctagctctggaagcaccccagcccctctagtctgccctcacccctgaccctgaccctccaccctgaccccgtcctaacccctgacctttgtgcccttccagagagaagggcagaagtgcccacagcccaccccagcccctcacccaggccagccggccagttccaaaccctggtggttggtgtcgtgggcggcctgctgggcagcctggtgctgctagtctgggtcctggccgtcatctgctcccgggccgcacgaggtaacgtcatcccagcccctcggcctgccctgccctaaccctgctggcggccctcactcccgcctccccttcctccacccttccctcaccccaccccacctccccccatctccccgccaggctaagtccctgatgaaggcccctggactaagaccccccacctaggagcacggctcagggtcggcctggtgaccccaagtgtgtttctctgcagggacaataggagccaggcgcaccggccagcccctggtgagtctcactcttttcctgcatgatccactgtgccttccttcctgggtgggcagaggtggaaggacaggctgggaccacacggcctgcaggactcacattctattatagccaggaccccacctccccagcccccaggcagcaacctcaatccctaaagccatgatctggggccccagcccacctgcggtctccgggggtgcccggcccatgtgtgtgcctgcctgcggtctccaggggtgcctggcccacgcgtgtgcccgcctgcggtctctgggggtgcccggcccacatatgtgcctgcctgcggtctccaggtgtgcccggcccatgcgtgtgcccacctgcgagggcgtggggtgggcttggtcatttcttatcttacattggagacaggagagcttgaaaagtcacattttggaatcctaaatctgcaagaatgccagggacatttcagagggggacattgagccagagaggaggggtggtgtccccagatcacacagagggcagtggtgggacagctcagggtaagcagctcgtagtggggggcccaggttcggtgccggtactgcagccaggctgtggagccgcgggcctccttcctgcggtgggccgtggggctgactccctctccctttctcctcaaagaaggaggacccctcagccgtgcctgtgttctctgtggactatggggagctggatttccagtggcgagagaagaccccggagccccccgtgccctgtgtccctgagcagacggagtaatgcatgaacagagaaacaggagaatatgggccaaacaggatatctgtggtaagcagttcctgccccggctcagggccaagaacagttggaacagcagaatatgggccaaacaggatatctgtggtaagcagttcctgccccggctcagggccaagaacagatggtccccagatgcggtcccgccctcagcagtttctagagaaccatcagatgtttccagggtgccccaaggacctgaaatgaccctgtgccttatttgaactaaccaatcagttcgcttctcgcttctgttcgcgcgcttctgctccccgagctctatataagcagagctcgtttagtgaaccgtcagatcgcctggagacgccatccacgctgttttgacttccatagaaggatctcgaggccaccatggctagcgagctgattaaggagaacatgcacatgaagctgtacatggagggcaccgtggacaaccatcacttcaagtgcacatccgagggcgaaggcaagccctacgagggcacccagaccatgagaatcaaggtggtcgagggcggccctctccccttcgccttcgacatcctggctactagcttcctctacggcagcaagaccttcatcaaccacacccagggcatccccgacttcttcaagcagtccttccctgagggcttcacatgggagagagtcaccacatacgaggacgggggcgtgctgaccgctacccaggacaccagcctccaggacggctgcctcatctacaacgtcaagatcagaggggtgaacttcacatccaacggccctgtgatgcagaagaaaacactcggctgggaggccttcaccgagacgctgtaccccgctgacggcggcctggaaggcagaaacgacatggccctgaagctcgtgggcgggagccatctgatcgcaaacatcaagaccacatatagatccaagaaacccgctaagaacctcaagatgcctggcgtctactatgtggactacagactggaaagaatcaaggaggccaacaacgagacctacgtcgagcagcacgaggtggcagtggccagatactgcgacctccctagcaaactggggcacaagctaaattgaaagctttgctttatttgtgaaatttgtgatgctattgctttatttgtaaccattataagctgcaataaacaagtttaacaacaacaattgcattcattttatgtttcaggttcagggggaggtgtgggaggttttttaaagtcgacccaccattgtctttcctagcggaatgggcacctcatcccccgcccgcaggggctcagctgacggccctcggagtgcccagccactgaggcctgaggatggacactgctcttggcccctctgaccggcttccttggccaccagtgttctgcagaccctccaccatgagcccgggtcagcgcatttcctcaggagaagcaggcagggtgcaggccattgcaggccgtccaggggctgagctgcctgggggcgaccggggctccagcctgcacctgcaccaggcacagccccaccacaggactcatgtctcaatgcccacagtgagcccaggcagcaggtgtcaccgtcccctacagggagggccagatgcagtcactgcttcaggtcctgccagcacagagctgcctgcgtccagctccctgaatctctgctgctgctgctgctgctgctgctgctgcctgcggcccggggctgaaggcgccgtggccctgcctgacgccccggagcctcctgcctgaacttgggggctggttggagatggccttggagcagccaaggtgcccctggcagtggcatcccgaaacgccctggacgcagggcccaagactgggcacaggagtgggaggtacatggggctggggactccccaggagttatctgctccctgcaggcctagagaagtttcagggaaggtcagaagagctcctggctgtggtgggcagggcaggaaacccctccacctttacacatgcccaggcagcacctcaggccctttgtggggcagggaagctgaggcagtaagcgggcaggcagagctggaggcctttcaggcccagccagcactctggcctcctgccgccgcattccaccccagcccctcacaccactcgggagagggacatcctacggtcccaaggtcaggagggcagggctggggttgactcaggcccctcccagctgtggccacctgggtgttgggagggcagaagtgcaggcacctagggccccccatgtgcccaccctgggagctctccttggaacccattcctgaaattatttaaaggggttggccggactagttacgtagataagtagcatggcgggttaatcattaactacaaggaacccctagtgatggagttggccactccctctctgcgcgctcgctcgctcactgaggccgggcgaccaaaggtcgcccgacgcccgggctttgcccgggcggcctcagtgagcgagcgagcgcgccagctggcgtaatagcgaagaggcccgcaccgatcgcccttcccaacagttgcgcagcctgaatggcgaatggcgattccgttgcaatggctggcggtaatattgttctggatattaccagcaaggccgatagtttgagttcttctactcaggcaagtgatgttattactaatcaaagaagtattgcgacaacggttaatttgcgtgatggacagactcttttactcggtggcctcactgattataaaaacacttctcaggattctggcgtaccgttcctgtctaaaatccctttaatcggcctcctgtttagctcccgctctgattctaacgaggaaagcacgttatacgtgctcgtcaaagcaaccatagtacgcgccctgtagcggcgcattaagcgcggcgggtgtggtggttacgcgcagcgtgaccgctacacttgccagcgccctagcgcccgctcctttcgctttcttcccttcctttctcgccacgttcgccggctttccccgtcaagctctaaatcgggggctccctttagggttccgatttagtgctttacggcacctcgaccccaaaaaacttgattagggtgatggttcacgtagtgggccatcgccctgatagacggtttttcgccctttgacgttggagtccacgttctttaatagtggactcttgttccaaactggaacaacactcaaccctatctcggtctattcttttgatttataagggattttgccgatttcggcctattggttaaaaaatgagctgatttaacaaaaatttaacgcgaattttaacaaaatattaacgtttacaatttaaatatttgcttatacaatcttcctgtttttggggcttttctgattatcaaccggggtacatatgattgacatgctagttttacgattaccgttcatcgattctcttgtttgctccagactctcaggcaatgacctgatagcctttgtagagacctctcaaaaatagctaccctctccggcatgaatttatcagctagaacggttgaatatcatattgatggtgatttgactgtctccggcctttctcacccgtttgaatctttacctacacattactcaggcattgcatttaaaatatatgagggttctaaaaatttttatccttgcgttgaaataaaggcttctcccgcaaaagtattacagggtcataatgtttttggtacaaccgatttagctttatgctctgaggctttattgcttaattttgctaattctttgccttgcctgtatgatttattggatgttggaatcgcctgatgcggtattttctccttacgcatctgtgcggtatttcacaccgcatatggtgcactctcagtacaatctgctctgatgccgcatagttaagccagccccgacacccgccaacacccgctgacgcgccctgacgggcttgtctgctcccggcatccgcttacagacaagctgtgaccgtctccgggagctgcatgtgtcagaggttttcaccgtcatcaccgaaacgcgcgagacgaaagggcctcgtgatacgcctatttttataggttaatgtcatgataataatggtttcttagacgtcaggtggcacttttcggggaaatgtgcgcggaacccctatttgtttatttttctaaatacattcaaatatgtatccgctcatgagacaataaccctgataaatgcttcaataatattgaaaaaggaagagtatgagtattcaacatttccgtgtcgcccttattcccttttttgcggcattttgccttcctgtttttgctcacccagaaacgctggtgaaagtaaaagatgctgaagatcagttgggtgcacgagtgggttacatcgaactggatctcaacagcggtaagatccttgagagttttcgccccgaagaacgttttccaatgatgagcacttttaaagttctgctatgtggcgcggtattatcccgtattgacgccgggcaagagcaactcggtcgccgcatacactattctcagaatgacttggttgagtactcaccagtcacagaaaagcatcttacggatggcatgacagtaagagaattatgcagtgctgccataaccatgagtgataacactgcggccaacttacttctgacaacgatcggaggaccgaaggagctaaccgcttttttgcacaacatgggggatcatgtaactcgccttgatcgttgggaaccggagctgaatgaagccataccaaacgacgagcgtgacaccacgatgcctgtagcaatggcaacaacgttgcgcaaactattaactggcgaactacttactctagcttcccggcaacaattaatagactggatggaggcggataaagttgcaggaccacttctgcgctcggcccttccggctggctggtttattgctgataaatctggagccggtgagcgtgggtctcgcggtatcattgcagcactggggccagatggtaagccctcccgtatcgtagttatctacacgacggggagtcaggcaactatggatgaacgaaatagacagatcgctgagataggtgcctcactgattaagcattggtaactgtcagaccaagtttactcatatatactttagattgatttaaaacttcatttttaatttaaaaggatctaggtgaagatcctttttgataatctcatgaccaaaatcccttaacgtgagttttcgttccactgagcgtcagaccccgtagaaaagatcaaaggatcttcttgagatcctttttttctgcgcgtaatctgctgcttgcaaacaaaaaaaccaccgctaccagcggtggtttgtttgccggatcaagagctaccaactctttttccgaaggtaactggcttcagcagagcgcagataccaaatactgtccttctagtgtagccgtagttaggccaccacttcaagaactctgtagcaccgcctacatacctcgctctgctaatcctgttaccagtggctgctgccagtggcgataagtcgtgtcttaccgggttggactcaagacgatagttaccggataaggcgcagcggtcgggctgaacggggggttcgtgcacacagcccagcttggagcgaacgacctacaccgaactgagatacctacagcgtgagctatgagaaagcgccacgcttcccgaagggagaaaggcggacaggtatccggtaagcggcagggtcggaacaggagagcgcacgagggagcttccagggggaaacgcctggtatctttatagtcctgtcgggtttcgccacctctgacttgagcgtcgatttttgtgatgctcgtcaggggggcggagcctatggaaaaacgccagcaacgcggcctttttacggttcctggccttttgctggccttttgctcacatgttctttcctgcgttatcccctgattctgtggataaccgtattaccgcctttgagtgagctgataccgctcgccgcagccgaacgaccgagcgcagcgagtcagtgagcgaggaagcggaagagcgcccaatacgcaaaccgcctctccccgcgcgttggccgattcattaatg

SEQ ID NO: 49 - DNA, 1325 bp, Homo sapiens
  source 1..1325: mol_type = unassigned DNA
agtccagggctctgtcctgcacctggggaatggtgaccggcatctctgtcctctagctctggaagcaccccagcccctctagtctgccctcacccctgaccctgaccctccaccctgaccccgtcctaacccctgacctttgtgcccttccagagagaagggcagaagtgcccacagcccaccccagcccctcacccaggccagccggccagttccaaaccctggtggttggtgtcgtgggcggcctgctgggcagcctggtgctgctagtctgggtcctggccgtcatctgctcccgggccgcacgaggtaacgtcatcccagcccctcggcctgccctgccctaaccctgctggcggccctcactcccgcctccccttcctccacccttccctcaccccaccccacctccccccatctccccgccaggctaagtccctgatgaaggcccctggactaagaccccccacctaggagcacggctcagggtcggcctggtgaccccaagtgtgtttctctgcagggacaataggagccaggcgcaccggccagcccctggtgagtctcactcttttcctgcatgatccactgtgccttccttcctgggtgggcagaggtggaaggacaggctgggaccacacggcctgcaggactcacattctattatagccaggaccccacctccccagcccccaggcagcaacctcaatccctaaagccatgatctggggccccagcccacctgcggtctccgggggtgcccggcccatgtgtgtgcctgcctgcggtctccaggggtgcctggcccacgcgtgtgcccgcctgcggtctctgggggtgcccggcccacatatgtgcctgcctgcggtctccaggtgtgcccggcccatgcgtgtgcccacctgcgagggcgtggggtgggcttggtcatttcttatcttacattggagacaggagagcttgaaaagtcacattttggaatcctaaatctgcaagaatgccagggacatttcagagggggacattgagccagagaggaggggtggtgtccccagatcacacagagggcagtggtgggacagctcagggtaagcagctcgtagtggggggcccaggttcggtgccggtactgcagccaggctgtggagccgcgggcctccttcctgcggtgggccgtggggctgactccctctccctttctcctcaaagaaggaggacccctcagccgtgcctgtgttctctgtggactatggggagctggatttccagtggcgagagaagaccccggagccccccgtgccctgtgtccctgagcagacggagta

SEQ ID NO: 50 - DNA, 1072 bp, Homo sapiens
  source 1..1072: mol_type = unassigned DNA
ccaccattgtctttcctagcggaatgggcacctcatcccccgcccgcaggggctcagccgacggccctcggagtgcccagccactgaggcctgaggatggacactgctcttggcccctctgaccggcttccttggccaccagtgttctgcagaccctccaccatgagcccgggtcagcgcatttcctcaggagaagcaggcagggtgcaggccattgcaggccgtccaggggctgagctgcctgggggcgaccggggctccagcctgcacctgcaccaggcacagccccaccacaggactcatgtctcaatgcccacagtgagcccaggcagcaggtgtcaccgtcccctacagggagggccagatgcagtcactgcttcaggtcctgccagcacagagctgcctgcgtccagctccctgaatctctgctgctgctgctgctgctgctgctgctgcctgcggcccggggctgaaggcgccgtggccctgcctgacgccccggagcctcctgcctgaacttgggggctggttggagatggccttggagcagccaaggtgcccctggcagtggcatcccgaaacgccctggacgcagggcccaagactgggcacaggagtgggaggtacatggggctggggactccccaggagttatctgctccctgcaggcctagagaagtttcagggaaggtcagaagagctcctggctgtggtgggcagggcaggaaacccctccacctttacacatgcccaggcagcacctcaggccctttgtggggcagggaagctgaggcagtaagcgggcaggcagagctggaggcctttcaggcccagccagcactctggcctcctgccgccgcattccaccccagcccctcacaccactcgggagagggacatcctacggtcccaaggtcaggagggcagggctggggttgactcaggcccctcccagctgtggccacctgggtgttgggagggcagaagtgcaggcacctagggccccccatgtgcccaccctgggagctctccttggaacccattcctgaaattatttaaaggggttggccgg

SEQ ID NO: 51 - DNA, 7880 bp, synthetic construct
  misc_feature 1..7880: note = Synthesized rAAV PD-1 Exon5_MND-PD-1-CD28 Switch Receptor construct
  source 1..7880: mol_type = other DNA
cagctgcgcgctcgctcgctcactgaggccgcccgggcaaagcccgggcgtcgggcgacctttggtcgcccggcctcagtgagcgagcgagcgcgcagagagggagtggccaactccatcactaggggttccttgtagttaatgattaacccgccatgctacttatctacgtagaattcagtccagggctctgtcctgcacctggggaatggtgaccggcatctctgtcctctagctctggaagcaccccagcccctctagtctgccctcacccctgaccctgaccctccaccctgaccccgtcctaacccctgacctttgtgcccttccagagagaagggcagaagtgcccacagcccaccccagcccctcacccaggccagccggccagttccaaaccctggtggttggtgtcgtgggcggcctgctgggcagcctggtgctgctagtctgggtcctggccgtcatctgctcccgggccgcacgaggtaacgtcatcccagcccctcggcctgccctgccctaaccctgctggcggccctcactcccgcctccccttcctccacccttccctcaccccaccccacctccccccatctccccgccaggctaagtccctgatgaaggcccctggactaagaccccccacctaggagcacggctcagggtcggcctggtgaccccaagtgtgtttctctgcagggacaataggagccaggcgcaccggccagcccctggtgagtctcactcttttcctgcatgatccactgtgccttccttcctgggtgggcagaggtggaaggacaggctgggaccacacggcctgcaggactcacattctattatagccaggaccccacctccccagcccccaggcagcaacctcaatccctaaagccatgatctggggccccagcccacctgcggtctccgggggtgcccggcccatgtgtgtgcctgcctgcggtctccaggggtgcctggcccacgcgtgtgcccgcctgcggtctctgggggtgcccggcccacatatgtgcctgcctgcggtctccaggtgtgcccggcccatgcgtgtgcccacctgcgagggcgtggggtgggcttggtcatttcttatcttacattggagacaggagagcttgaaaagtcacattttggaatcctaaatctgcaagaatgccagggacatttcagagggggacattgagccagagaggaggggtggtgtccccagatcacacagagggcagtggtgggacagctcagggtaagcagctcatagtggggggcccaggttcggtgccggtactgcagccaggctgtggagccgcgggcctccttcctgcggtgggccgtggggctgactccctctccctttctcctcaaagaaggaggacccctcagccgtgcctgtgttctctgtggactatggggagctggatttccagtggcgagagaagaccccggagccccccgtgccctgtgtccctgagcagacggagtaatgcatgaacagagaaacaggagaatatgggccaaacaggatatctgtggtaagcagttcctgccccggctcagggccaagaacagttggaacagcagaatatgggccaaacaggatatctgtggtaagcagttcctgccccggctcagggccaagaacagatggtccccagatgcggtcccgccctcagcagtttctagagaaccatcagatgtttccagggtgccccaaggacctgaaatgaccctgtgccttatttgaactaaccaatcagttcgcttctcgcttctgttcgcgcgcttctgctccccgagctctatataagcagagctcgtttagtgaaccgtcagatcgcctggagacgccatccacgctgttttgacttccatagaaggatctcgaggccaccatgcagatcccgcaagcgccctggccagtcgtctgggcggtgctacaactgggctggcggccaggatggttcttagactccccagacaggccctggaacccccccaccttctccccagccctgctcgtggtgaccgaaggggacaacgccaccttcacctgcagcttctccaacacatcggagagcttcgtgctaaactggtaccgcatgagccccagcaaccagacggacaagctggccgccttccccgaggaccgcagccagcccggccaggactgccgcttccgtgtcacacaactgcccaacgggcgtgacttccacatgagcgtggtcagggcccggcgcaatgacagcggcacctacctctgtggggccatctccctggcccccaaggcgcagatcaaagagagcctgcgggcagagctcagggtgacagagagaagggcagaagtgcccacagcccaccccagcccctcacccaggccagccggccagttccaaaccctggtggttggtgtcgtgggcggcctgctgggcagcctggtgctgctagtctgggtcctggccgtcatcaggagtaagaggagcaggctcctgcacagtgactacatgaacatgactccccgccgccccgggcccacccgcaagcattaccagccctatgccccaccacgcgacttcgcagcctatcgctccggtgagggcagaggaagtcttctaacatgcggtgacgtggaggagaatccgggccctgtgagcaagggcgaggaggataactccgccatcatcaaggagttcctgcgcttcaaggtgcacatggagggctccgtgaacggccacgagttcgagatcgagggcgagggcgagggccgcccctacgagggcacccagaccgccaagctgaaggtgaccaagggtggccccctgcccttcgcctgggacatcctgtcccctcagttcatgtacggctccaaggcctacgtgaagcaccccgccgacatccccgactacttgaagctgtccttccccgagggcttcaagtgggagcgcgtgatgaacttcgaggacggcggcgtggtgaccgtgacccaggactcctctctgcaggacggcgagttcatctacaaggtgaagctgcgcggcaccaacttcccctccgacggccccgtaatgcagaagaagaccatgggctgggaggcctcctccgagcggatgtaccccgaggacggcgccctgaagggcgagatcaagcagaggctgaagctgaaggacggcggccactacgacgctgaggtcaagaccacctacaaggccaagaagcccgtgcagctgcccggcgcctacaacgtcaacatcaagttggacatcacctcccacaacgaggactacaccatcgtggaacagtacgaacgcgccgagggccgccactccaccggcggcatggacgagctgtacaagtgatgaaagctttgctttatttgtgaaatttgtgatgctattgctttatttgtaaccattataagctgcaataaacaagtttaacaacaacaattgcattcattttatgtttcaggttcagggggaggtgtgggaggttttttaaagtcgacgtggccctgcctgacgccccggagcctcctgcctgaacttgggggctggttggagatggccttggagcagccaaggtgcccctggcagtggcatcccgaaacgccctggacgcagggcccaagactgggcacaggagtgggaggtacatggggctggggactccccaggagttatctgctccctgcaggcctagagaagtttcagggaaggtcagaagagctcctggctgtggtgggcagggcaggaaacccctccacctttacacatgcccaggcagcacctcaggccctttgtggggcagggaagctgaggcagtaagcgggcaggcagagctggaggcctttcaggcccagccagcactctggcctcctgccgccgcattccaccccagcccctcacaccactcgggagagggacatcctacggtcccaaggtcaggagggcagggctggggttgactcaggcccctcccagctgtggccacctgggtgttgggagggcagaagtgcaggcacctagggccccccatgtgcccaccctgggagctctccttggaacccattcctgaaattatttaaaggggttggccggactagttacgtagataagtagcatggcgggttaatcattaactacaaggaacccctagtgatggagttggccactccctctctgcgcgctcgctcgctcactgaggccgggcgaccaaaggtcgcccgacgcccgggctttgcccgggcggcctcagtgagcgagcgagcgcgccagctggcgtaatagcgaagaggcccgcaccgatcgcccttcccaacagttgcgcagcctgaatggcgaatggcgattccgttgcaatggctggcggtaatattgttctggatattaccagcaaggccgatagtttgagttcttctactcaggcaagtgatgttattactaatcaaagaagtattgcgacaacggttaatttgcgtgatggacagactcttttactcggtggcctcactgattataaaaacacttctcaggattctggcgtaccgttcctgtctaaaatccctttaatcggcctcctgtttagctcccgctctgattctaacgaggaaagcacgttatacgtgctcgtcaaagcaaccatagtacgcgccctgtagcggcgcattaagcgcggcgggtgtggtggttacgcgcagcgtgaccgctacacttgccagcgccctagcgcccgctcctttcgctttcttcccttcctttctcgccacgttcgccggctttccccgtcaagctctaaatcgggggctccctttagggttccgatttagtgctttacggcacctcgaccccaaaaaacttgattagggtgatggttcacgtagtgggccatcgccctgatagacggtttttcgccctttgacgttggagtccacgttctttaatagtggactcttgttccaaactggaacaacactcaaccctatctcggtctattcttttgatttataagggattttgccgatttcggcctattggttaaaaaatgagctgatttaacaaaaatttaacgcgaattttaacaaaatattaacgtttacaatttaaatatttgcttatacaatcttcctgtttttggggcttttctgattatcaaccggggtacatatgattgacatgctagttttacgattaccgttcatcgattctcttgtttgctccagactctcaggcaatgacctgatagcctttgtagagacctctcaaaaatagctaccctctccggcatgaatttatcagctagaacggttgaatatcatattgatggtgatttgactgtctccggcctttctcacccgtttgaatctttacctacacattactcaggcattgcatttaaaatatatgagggttctaaaaatttttatccttgcgttgaaataaaggcttctcccgcaaaagtattacagggtcataatgtttttggtacaaccgatttagctttatgctctgaggctttattgcttaattttgctaattctttgccttgcctgtatgatttattggatgttggaatcgcctgatgcggtattttctccttacgcatctgtgcggtatttcacaccgcatatggtgcactctcagtacaatctgctctgatgccgcatagttaagccagccccgacacccgccaacacccgctgacgcgccctgacgggcttgtctgctcccggcatccgcttacagacaagctgtgaccgtctccgggagctgcatgtgtcagaggttttcaccgtcatcaccgaaacgcgcgagacgaaagggcctcgtgatacgcctatttttataggttaatgtcatgataataatggtttcttagacgtcaggtggcacttttcggggaaatgtgcgcggaacccctatttgtttatttttctaaatacattcaaatatgtatccgctcatgagacaataaccctgataaatgcttcaataatattgaaaaaggaagagtatgagtattcaacatttccgtgtcgcccttattcccttttttgcggcattttgccttcctgtttttgctcacccagaaacgctggtgaaagtaaaagatgctgaagatcagttgggtgcacgagtgggttacatcgaactggatctcaacagcggtaagatccttgagagttttcgccccgaagaacgttttccaatgatgagcacttttaaagttctgctatgtggcgcggtattatcccgtattgacgccgggcaagagcaactcggtcgccgcatacactattctcagaatgacttggttgagtactcaccagtcacagaaaagcatcttacggatggcatgacagtaagagaattatgcagtgctgccataaccatgagtgataacactgcggccaacttacttctgacaacgatcggaggaccgaaggagctaaccgcttttttgcacaacatgggggatcatgtaactcgccttgatcgttgggaaccggagctgaatgaagccataccaaacgacgagcgtgacaccacgatgcctgtagcaatggcaacaacgttgcgcaaactattaactggcgaactacttactctagcttcccggcaacaattaatagactggatggaggcggataaagttgcaggaccacttctgcgctcggcccttccggctggctggtttattgctgataaatctggagccggtgagcgtgggtctcgcggtatcattgcagcactggggccagatggtaagccctcccgtatcgtagttatctacacgacggggagtcaggcaactatggatgaacgaaatagacagatcgctgagataggtgcctcactgattaagcattggtaactgtcagaccaagtttactcatatatactttagattgatttaaaacttcatttttaatttaaaaggatctaggtgaagatcctttttgataatctcatgaccaaaatcccttaacgtgagttttcgttccactgagcgtcagaccccgtagaaaagatcaaaggatcttcttgagatcctttttttctgcgcgtaatctgctgcttgcaaacaaaaaaaccaccgctaccagcggtggtttgtttgccggatcaagagctaccaactctttttccgaaggtaactggcttcagcagagcgcagataccaaatactgtccttctagtgtagccgtagttaggccaccacttcaagaactctgtagcaccgcctacatacctcgctctgctaatcctgttaccagtggctgctgccagtggcgataagtcgtgtcttaccgggttggactcaagacgatagttaccggataaggcgcagcggtcgggctgaacggggggttcgtgcacacagcccagcttggagcgaacgacctacaccgaactgagatacctacagcgtgagctatgagaaagcgccacgcttcccgaagggagaaaggcggacaggtatccggtaagcggcagggtcggaacaggagagcgcacgagggagcttccagggggaaacgcctggtatctttatagtcctgtcgggtttcgccacctctgacttgagcgtcgatttttgtgatgctcgtcaggggggcggagcctatggaaaaacgccagcaacgcggcctttttacggttcctggccttttgctggccttttgctcacatgttctttcctgcgttatcccctgattctgtggataaccgtattaccgcctttgagtgagctgataccgctcgccgcagccgaacgaccgagcgcagcgagtcagtgagcgaggaagcggaagagcgcccaatacgcaaaccgcctctccccgcgcgttggccgattcattaatg

SEQ ID NO: 52 - DNA, 7593 bp, synthetic construct
  misc_feature 1..7593: note = Synthesized rAAV PD-1 Exon5_MND-BFP_distal 5'-Homology Arm construct
  source 1..7593: mol_type = other DNA
cagctgcgcgctcgctcgctcactgaggccgcccgggcaaagcccgggcgtcgggcgacctttggtcgcccggcctcagtgagcgagcgagcgcgcagagagggagtggccaactccatcactaggggttccttgtagttaatgattaacccgccatgctacttatctacgtagaattcggccccactgcccactgcccagggcagcaatgcccataccacgtggtcccagctccgagcttgtcctgaaaagggggcaaagactggaccctgagcctgccaaggggccacactcctcccagggctggggtctccatgggcagccccccacccacccagaccagttacactcccctgtgccagagcagtgcagacaggaccaggccaggatgcccaagggtcaggggctggggatgggtagcccccaaacagccctttctgggggactggcctcaacggggaagggggtgaaggctcttagtaggaaatcagggagacccaagtcagagccaggcgctgtgcagaagctgcagcctcacgtagaaggaagagcctctgcagtggaggccagtgcccatccccgggtggcagaggccccagcagagacttctcaatgacattccagctggggtggcccttccagagcccttgctgcccgagggatgtgagcaggtggccggggaggctttgtggggccacccagccccttcctcacctctctccatctctcagactccccagacaggccctggaacccccccaccttctccccagccctgctcgtggtgaccgaaggggacaacgccaccttcacctgcagcttctccaacacatcggagagcttcgtgctaaactggtaccgcatgagccccagcaaccagacggacaagctggccgccttccccgaggaccgcagccagcccggccaggactgccgcttccgtgtcacacaactgcccaacgggcgtgacttccacatgagcgtggtcagggcccggcgcaatgacagcggcacctacctctgtggggccatctccctggcccccaaggcgcagatcaaagagagcctgcgggcagagctcagggtgacaggtgcggcctcggaggccccggggcaggggtgagctgagccggtcctggggtgggtgtcccctcctgcacaggatcaggagctccagggtcgtagggcagggaccccccagctccagtccagggctctgtcctgcacctggggaatggtgaccggcatctctgtcctctagctctggaagcaccccagcccctctagtctgccctcacccctgaccctgaccctccaccctgaccccgtcctaacccctgacctttgtgcccttccagagagaagggcagaagtgcccacagcccaccccagcccctcacccaggccagccggccagttccaaaccctggtggttggtgtcgtgggcggcctgctgggcagcctggtgctgctagtctgggtcctggccgtcatctatgcatgaacagagaaacaggagaatatgggccaaacaggatatctgtggtaagcagttcctgccccggctcagggccaagaacagttggaacagcagaatatgggccaaacaggatatctgtggtaagcagttcctgccccggctcagggccaagaacagatggtccccagatgcggtcccgccctcagcagtttctagagaaccatcagatgtttccagggtgccccaaggacctgaaatgaccctgtgccttatttgaactaaccaatcagttcgcttctcgcttctgttcgcgcgcttctgctccccgagctctatataagcagagctcgtttagtgaaccgtcagatcgcctggagacgccatccacgctgttttgacttccatagaaggatctcgaggccaccatggctagcgagctgattaaggagaacatgcacatgaagctgtacatggagggcaccgtggacaaccatcacttcaagtgcacatccgagggcgaaggcaagccctacgagggcacccagaccatgagaatcaaggtggtcgagggcggccctctccccttcgccttcgacatcctggctactagcttcctctacggcagcaagaccttcatcaaccacacccagggcatccccgacttcttcaagcagtccttccctgagggcttcacatgggagagagtcaccacatacgaggacgggggcgtgctgaccgctacccaggacaccagcctccaggacggctgcctcatctacaacgtcaagatcagaggggtgaacttcacatccaacggccctgtgatgcagaagaaaacactcggctgggaggccttcaccgagacgctgtaccccgctgacggcggcctggaaggcagaaacgacatggccctgaagctcgtgggcgggagccatctgatcgcaaacatcaagaccacatatagatccaagaaacccgctaagaacctcaagatgcctggcgtctactatgtggactacagactggaaagaatcaaggaggccaacaacgagacctacgtcgagcagcacgaggtggcagtggccagatactgcgacctccctagcaaactggggcacaagctaaattgaaagctttgctttatttgtgaaatttgtgatgctattgctttatttgtaaccattataagctgcaataaacaagtttaacaacaacaattgcattcattttatgtttcaggttcagggggaggtgtgggaggttttttaaagtcgacccaccattgtctttcctagcggaatgggcacctcatcccccgcccgcaggggctcagctgacggccctcggagtgcccagccactgaggcctgaggatggacactgctcttggcccctctgaccggcttccttggccaccagtgttctgcagaccctccaccatgagcccgggtcagcgcatttcctcaggagaagcaggcagggtgcaggccattgcaggccgtccaggggctgagctgcctgggggcgaccggggctccagcctgcacctgcaccaggcacagccccaccacaggactcatgtctcaatgcccacagtgagcccaggcagcaggtgtcaccgtcccctacagggagggccagatgcagtcactgcttcaggtcctgccagcacagagctgcctgcgtccagctccctgaatctctgctgctgctgctgctgctgctgctgctgcctgcggcccggggctgaaggcgccgtggccctgcctgacgccccggagcctcctgcctgaacttgggggctggttggagatggccttggagcagccaaggtgcccctggcagtggcatcccgaaacgccctggacgcagggcccaagactgggcacaggagtgggaggtacatggggctggggactccccaggagttatctgctccctgcaggcctagagaagtttcagggaaggtcagaagagctcctggctgtggtgggcagggcaggaaacccctccacctttacacatgcccaggcagcacctcaggccctttgtggggcagggaagctgaggcagtaagcgggcaggcagagctggaggcctttcaggcccagccagcactctggcctcctgccgccgcattccaccccagcccctcacaccactcgggagagggacatcctacggtcccaaggtcaggagggcagggctggggttgactcaggcccctcccagctgtggccacctgggtgttgggagggcagaagtgcaggcacctagggccccccatgtgcccaccctgggagctctccttggaacccattcctgaaattatttaaaggggttggccggactagttacgtagataagtagcatggcgggttaatcattaactacaaggaacccctagtgatggagttggccactccctctctgcgcgctcgctcgctcactgaggccgggcgaccaaaggtcgcccgacgcccgggctttgcccgggcggcctcagtgagcgagcgagcgcgccagctggcgtaatagcgaagaggcccgcaccgatcgcccttcccaacagttgcgcagcctgaatggcgaatggcgattccgttgcaatggctggcggtaatattgttctggatattaccagcaaggccgatagtttgagttcttctactcaggcaagtgatgttattactaatcaaagaagtattgcgacaacggttaatttgcgtgatggacagactcttttactcggtggcctcactgattataaaaacacttctcaggattctggcgtaccgttcctgtctaaaatccctttaatcggcctcctgtttagctcccgctctgattctaacgaggaaagcacgttatacgtgctcgtcaaagcaaccatagtacgcgccctgtagcggcgcattaagcgcggcgggtgtggtggttacgcgcagcgtgaccgctacacttgccagcgccctagcgcccgctcctttcgctttcttcccttcctttctcgccacgttcgccggctttccccgtcaagctctaaatcgggggctccctttagggttccgatttagtgctttacggcacctcgaccccaaaaaacttgattagggtgatggttcacgtagtgggccatcgccctgatagacggtttttcgccctttgacgttggagtccacgttctttaatagtggactcttgttccaaactggaacaacactcaaccctatctcggtctattcttttgatttataagggattttgccgatttcggcctattggttaaaaaatgagctgatttaacaaaaatttaacgcgaattttaacaaaatattaacgtttacaatttaaatatttgcttatacaatcttcctgtttttggggcttttctgattatcaaccggggtacatatgattgacatgctagttttacgattaccgttcatcgattctcttgtttgctccagactctcaggcaatgacctgatagcctttgtagagacctctcaaaaatagctaccctctccggcatgaatttatcagctagaacggttgaatatcatattgatggtgatttgactgtctccggcctttctcacccgtttgaatctttacctacacattactcaggcattgcatttaaaatatatgagggttctaaaaatttttatccttgcgttgaaataaaggcttctcccgcaaaagtattacagggtcataatgtttttggtacaaccgatttagctttatgctctgaggctttattgcttaattttgctaattctttgccttgcctgtatgatttattggatgttggaatcgcctgatgcggtattttctccttacgcatctgtgcggtatttcacaccgcatatggtgcactctcagtacaatctgctctgatgccgcatagttaagccagccccgacacccgccaacacccgctgacgcgccctgacgggcttgtctgctcccggcatccgcttacagacaagctgtgaccgtctccgggagctgcatgtgtcagaggttttcaccgtcatcaccgaaacgcgcgagacgaaagggcctcgtgatacgcctatttttataggttaatgtcatgataataatggtttcttagacgtcaggtggcacttttcggggaaatgtgcgcggaacccctatttgtttatttttctaaatacattcaaatatgtatccgctcatgagacaataaccctgataaatgcttcaataatattgaaaaaggaagagtatgagtattcaacatttccgtgtcgcccttattcccttttttgcggcattttgccttcctgtttttgctcacccagaaacgctggtgaaagtaaaagatgctgaagatcagttgggtgcacgagtgggttacatcgaactggatctcaacagcggtaagatccttgagagttttcgccccgaagaacgttttccaatgatgagcacttttaaagttctgctatgtggcgcggtattatcccgtattgacgccgggcaagagcaactcggtcgccgcatacactattctcagaatgacttggttgagtactcaccagtcacagaaaagcatcttacggatggcatgacagtaagagaattatgcagtgctgccataaccatgagtgataacactgcggccaacttacttctgacaacgatcggaggaccgaaggagctaaccgcttttttgcacaacatgggggatcatgtaactcgccttgatcgttgggaaccggagctgaatgaagccataccaaacgacgagcgtgacaccacgatgcctgtagcaatggcaacaacgttgcgcaaactattaactggcgaactacttactctagcttcccggcaacaattaatagactggatggaggcggataaagttgcaggaccacttctgcgctcggcccttccggctggctggtttattgctgataaatctggagccggtgagcgtgggtctcgcggtatcattgcagcactggggccagatggtaagccctcccgtatcgtagttatctacacgacggggagtcaggcaactatggatgaacgaaatagacagatcgctgagataggtgcctcactgattaagcattggtaactgtcagaccaagtttactcatatatactttagattgatttaaaacttcatttttaatttaaaaggatctaggtgaagatcctttttgataatctcatgaccaaaatcccttaacgtgagttttcgttccactgagcgtcagaccccgtagaaaagatcaaaggatcttcttgagatcctttttttctgcgcgtaatctgctgcttgcaaacaaaaaaaccaccgctaccagcggtggtttgtttgccggatcaagagctaccaactctttttccgaaggtaactggcttcagcagagcgcagataccaaatactgtccttctagtgtagccgtagttaggccaccacttcaagaactctgtagcaccgcctacatacctcgctctgctaatcctgttaccagtggctgctgccagtggcgataagtcgtgtcttaccgggttggactcaagacgatagttaccggataaggcgcagcggtcgggctgaacggggggttcgtgcacacagcccagcttggagcgaacgacctacaccgaactgagatacctacagcgtgagctatgagaaagcgccacgcttcccgaagggagaaaggcggacaggtatccggtaagcggcagggtcggaacaggagagcgcacgagggagcttccagggggaaacgcctggtatctttatagtcctgtcgggtttcgccacctctgacttgagcgtcgatttttgtgatgctcgtcaggggggcggagcctatggaaaaacgccagcaacgcggcctttttacggttcctggccttttgctggccttttgctcacatgttctttcctgcgttatcccctgattctgtggataaccgtattaccgcctttgagtgagctgataccgctcgccgcagccgaacgaccgagcgcagcgagtcagtgagcgaggaagcggaagagcgcccaatacgcaaaccgcctctccccgcgcgttggccgattcattaatg

SEQ ID NO: 53 - DNA, 6718 bp, synthetic construct
  misc_feature 1..6718: note = Synthesized rAAV PD-1 Exon1_MND-GFP construct
  source 1..6718: mol_type = other DNA
cagctgcgcgctcgctcgctcactgaggccgcccgggcaaagcccgggcgtcgggcgacctttggtcgcccggcctcagtgagcgagcgagcgcgcagagagggagtggccaactccatcactaggggttccttgtagttaatgattaacccgccatgctacttatctacgtaaggctgttgcaggcatcacacggtggaaagatctggaactgtggccatggtgtgaggccatccacaaggtggaagctttgagggggagccgattagccatggacagttgtcattcagtagggtcacctgtgccccagcgaagggggatgggccgggaaggcagaggccaggcacctgcccccagcaggggcagaggctgtgggcagccgggaggctcccagaggctccgacagaatgggagtggggttgagcccacccctcactgcagcccaggaacctgagcccagagggggccacccaccttccccaggcagggaggcccggcccccagggagatgggggggatgggggaggagaagggcctgcccccacccggcagcctcaggaggggcagctcgggcgggatatggaaagaggccacagcagtgagcagagacacagaggaggaaggggccctgagctggggagacccccacggggtagggcgtgggggccacgggcccacctcctccccatctcctctgtctccctgtctctgtctctctctccctcccccaccctctccccagtcctaccccctcctcacccctcctcccccagcactgcctctgtcactctcgcccacgtggatgtggaggaagagggggcgggagcaaggggcgggcaccctcccttcaacctgacctgggacagtttcccttccgctcacctccgcctgagcagtggagaaggcggcactctggtggggctgctccaacgcgtgaacagagaaacaggagaatatgggccaaacaggatatctgtggtaagcagttcctgccccggctcagggccaagaacagttggaacagcagaatatgggccaaacaggatatctgtggtaagcagttcctgccccggctcagggccaagaacagatggtccccagatgcggtcccgccctcagcagtttctagagaaccatcagatgtttccagggtgccccaaggacctgaaatgaccctgtgccttatttgaactaaccaatcagttcgcttctcgcttctgttcgcgcgcttctgctccccgagctctatataagcagagctcgtttagtgaaccgtcagatcgcctggagacgccatccacgctgttttgacttccatagaaggatctcgaggccaccatggtgagcaagggcgaggagctgttcaccggggtggtgcccatcctggtcgagctggacggcgacgtaaacggccacaagttcagcgtgtccggcgagggcgagggcgatgccacctacggcaagctgaccctgaagttcatctgcaccaccggcaagctgcccgtgccctggcccaccctcgtgaccaccctgacctacggcgtgcagtgcttcagccgctaccccgaccacatgaagcagcacgacttcttcaagtccgccatgcccgaaggctacgtccaggagcgcaccatcttcttcaaggacgacggcaactacaagacccgcgccgaggtgaagttcgagggcgacaccctggtgaaccgcatcgagctgaagggcatcgacttcaaggaggacggcaacatcctggggcacaagctggagtacaactacaacagccacaacgtctatatcatggccgacaagcagaagaacggcatcaaggtgaacttcaagatccgccacaacatcgaggacggcagcgtgcagctcgccgaccactaccagcagaacacccccatcggcgacggccccgtgctgctgcccgacaaccactacctgagcacccagtccgccctgagcaaagaccccaacgagaagcgcgatcacatggtcctgctggagttcgtgaccgccgccgggatcactctcggcatggacgagctgtacaagtaagcggccgcgctttatttgtgaaatttgtgatgctattgctttatttgtaaccattataagctgcaataaacaagttaacaacaacaattgcattcattttatgtttcaggttcagggggagatgtgggaggttttttaaagcctcaccggttctgggcggtgctacaactgggctggcggccaggatggttcttaggtaggtggggtcggcggtcaggtgtcccagagccaggggtctggagggaccttccaccctcagtccctggcaggtcggggggtgctgaggcgggcctggccctggcagcccaggggtcccggagcgaggggtctggagggacctttcactctcagtccctggcaggtcggggggtgctgtggcaggcccagccttggcccccagctctgccccttaccctgagctgtgtggctttgggcagctcgaactcctgggttcctctctgggccccaactcctcccctggcccaagtcccctctttgctcctgggcaggcaggacctctgtcccctctcagccggtccttggggctgcgtgtttctgtagaatgacgggtcaggctggccagaaccccaaaccttggccgtggggagtctgcgtggcggctctgccttgcccaggcatccttggtcctcactcgagttttcctaaggatgggatgagccccatgtgggactaaccttggctttacgacgtcaaagtttagatgagctggtgatatttttctcattatatccaaagtgtacctgttcgagtgaggacagttcttctgtctccaggatccctcctgggtggggattgtgcccgcctgggtctctgcccagattccagggctctccccgagccctgttcagaccatccgtgggggaggccttggcctcactcttacgtagataagtagcatggcgggttaatcattaactacaaggaacccctagtgatggagttggccactccctctctgcgcgctcgctcgctcactgaggccgggcgaccaaaggtcgcccgacgcccgggctttgcccgggcggcctcagtgagcgagcgagcgcgccagctggcgtaatagcgaagaggcccgcaccgatcgcccttcccaacagttgcgcagcctgaatggcgaatggcgattccgttgcaatggctggcggtaatattgttctggatattaccagcaaggccgatagtttgagttcttctactcaggcaagtgatgttattactaatcaaagaagtattgcgacaacggttaatttgcgtgatggacagactcttttactcggtggcctcactgattataaaaacacttctcaggattctggcgtaccgttcctgtctaaaatccctttaatcggcctcctgtttagctcccgctctgattctaacgaggaaagcacgttatacgtgctcgtcaaagcaaccatagtacgcgccctgtagcggcgcattaagcgcggcgggtgtggtggttacgcgcagcgtgaccgctacacttgccagcgccctagcgcccgctcctttcgctttcttcccttcctttctcgccacgttcgccggctttccccgtcaagctctaaatcgggggctccctttagggttccgatttagtgctttacggcacctcgaccccaaaaaacttgattagggtgatggttcacgtagtgggccatcgccctgatagacggtttttcgccctttgacgttggagtccacgttctttaatagtggactcttgttccaaactggaacaacactcaaccctatctcggtctattcttttgatttataagggattttgccgatttcggcctattggttaaaaaatgagctgatttaacaaaaatttaacgcgaattttaacaaaatattaacgtttacaatttaaatatttgcttatacaatcttcctgtttttggggcttttctgattatcaaccggggtacatatgattgacatgctagttttacgattaccgttcatcgattctcttgtttgctccagactctcaggcaatgacctgatagcctttgtagagacctctcaaaaatagctaccctctccggcatgaatttatcagctagaacggttgaatatcatattgatggtgatttgactgtctccggcctttctcacccgtttgaatctttacctacacattactcaggcattgcatttaaaatatatgagggttctaaaaatttttatccttgcgttgaaataaaggcttctcccgcaaaagtattacagggtcataatgtttttggtacaaccgatttagctttatgctctgaggctttattgcttaattttgctaattctttgccttgcctgtatgatttattggatgttggaatcgcctgatgcggtattttctccttacgcatctgtgcggtatttcacaccgcatatggtgcactctcagtacaatctgctctgatgccgcatagttaagccagccccgacacccgccaacacccgctgacgcgccctgacgggcttgtctgctcccggcatccgcttacagacaagctgtgaccgtctccgggagctgcatgtgtcagaggttttcaccgtcatcaccgaaacgcgcgagacgaaagggcctcgtgatacgcctatttttataggttaatgtcatgataataatggtttcttagacgtcaggtggcacttttcggggaaatgtgcgcggaacccctatttgtttatttttctaaatacattcaaatatgtatccgctcatgagacaataaccctgataaatgcttcaataatattgaaaaaggaagagtatgagtattcaacatttccgtgtcgcccttattcccttttttgcggcattttgccttcctgtttttgctcacccagaaacgctggtgaaagtaaaagatgctgaagatcagttgggtgcacgagtgggttacatcgaactggatctcaacagcggtaagatccttgagagttttcgccccgaagaacgttttccaatgatgagcacttttaaagttctgctatgtggcgcggtattatcccgtattgacgccgggcaagagcaactcggtcgccgcatacactattctcagaatgacttggttgagtactcaccagtcacagaaaagcatcttacggatggcatgacagtaagagaattatgcagtgctgccataaccatgagtgataacactgcggccaacttacttctgacaacgatcggaggaccgaaggagctaaccgcttttttgcacaacatgggggatcatgtaactcgccttgatcgttgggaaccggagctgaatgaagccataccaaacgacgagcgtgacaccacgatgcctgtagcaatggcaacaacgttgcgcaaactattaactggcgaactacttactctagcttcccggcaacaattaatagactggatggaggcggataaagttgcaggaccacttctgcgctcggcccttccggctggctggtttattgctgataaatctggagccggtgagcgtgggtctcgcggtatcattgcagcactggggccagatggtaagccctcccgtatcgtagttatctacacgacggggagtcaggcaactatggatgaacgaaatagacagatcgctgagataggtgcctcactgattaagcattggtaactgtcagaccaagtttactcatatatactttagattgatttaaaacttcatttttaatttaaaaggatctaggtgaagatcctttttgataatctcatgaccaaaatcccttaacgtgagttttcgttccactgagcgtcagaccccgtagaaaagatcaaaggatcttcttgagatcctttttttctgcgcgtaatctgctgcttgcaaacaaaaaaaccaccgctaccagcggtggtttgtttgccggatcaagagctaccaactctttttccgaaggtaactggcttcagcagagcgcagataccaaatactgtccttctagtgtagccgtagttaggccaccacttcaagaactctgtagcaccgcctacatacctcgctctgctaatcctgttaccagtggctgctgccagtggcgataagtcgtgtcttaccgggttggactcaagacgatagttaccggataaggcgcagcggtcgggctgaacggggggttcgtgcacacagcccagcttggagcgaacgacctacaccgaactgagatacctacagcgtgagctatgagaaagcgccacgcttcccgaagggagaaaggcggacaggtatccggtaagcggcagggtcggaacaggagagcgcacgagggagcttccagggggaaacgcctggtatctttatagtcctgtcgggtttcgccacctctgacttgagcgtcgatttttgtgatgctcgtcaggggggcggagcctatggaaaaacgccagcaacgcggcctttttacggttcctggccttttgctggccttttgctcacatgttctttcctgcgttatcccctgattctgtggataaccgtattaccgcctttgagtgagctgataccgctcgccgcagccgaacgaccgagcgcagcgagtcagtgagcgaggaagcggaagagcgcccaatacgcaaaccgcctctccccgcgcgttggccgattcattaatg

SEQ ID NO: 54 - DNA, 756 bp, Homo sapiens
  source 1..756: mol_type = unassigned DNA
aggctgttgcaggcatcacacggtggaaagatctggaactgtggccatggtgtgaggccatccacaaggtggaagctttgagggggagccgattagccatggacagttgtcattcagtagggtcacctgtgccccagcgaagggggatgggccgggaaggcagaggccaggcacctgcccccagcaggggcagaggctgtgggcagccgggaggctcccagaggctccgacagaatgggagtggggttgagcccacccctcactgcagcccaggaacctgagcccagagggggccacccaccttccccaggcagggaggcccggcccccagggagatgggggggatgggggaggagaagggcctgcccccacccggcagcctcaggaggggcagctcgggcgggatatggaaagaggccacagcagtgagcagagacacagaggaggaaggggccctgagctggggagacccccacggggtagggcgtgggggccacgggcccacctcctccccatctcctctgtctccctgtctctgtctctctctccctcccccaccctctccccagtcctaccccctcctcacccctcctcccccagcactgcctctgtcactctcgcccacgtggatgtggaggaagagggggcgggagcaaggggcgggcaccctcccttcaacctgacctgggacagtttcccttccgctcacctccgcctgagcagtggagaaggcggcactctggtggggctgctcca

SEQ ID NO: 55 - DNA, 750 bp, Homo sapiens
  source 1..750: mol_type = unassigned DNA
tctgggcggtgctacaactgggctggcggccaggatggttcttaggtaggtggggtcggcggtcaggtgtcccagagccaggggtctggagggaccttccaccctcagtccctggcaggtcggggggtgctgaggcgggcctggccctggcagcccaggggtcccggagcgaggggtctggagggacctttcactctcagtccctggcaggtcggggggtgctgtggcaggcccagccttggcccccagctctgccccttaccctgagctgtgtggctttgggcagctcgaactcctgggttcctctctgggccccaactcctcccctggcccaagtcccctctttgctcctgggcaggcaggacctctgtcccctctcagccggtccttggggctgcgtgtttctgtagaatgacgggtcaggctggccagaaccccaaaccttggccgtggggagtctgcgtggcggctctgccttgcccaggcatccttggtcctcactcgagttttcctaaggatgggatgagccccatgtgggactaaccttggctttacgacgtcaaagtttagatgagctggtgatatttttctcattatatccaaagtgtacctgttcgagtgaggacagttcttctgtctccaggatccctcctgggtggggattgtgcccgcctgggtctctgcccagattccagggctctccccgagccctgttcagaccatccgtgggggaggccttggcctcactct

SEQ ID NO: 56 - DNA, 7609 bp, synthetic construct
  misc_feature 1..7609: note = Synthesized rAAV PD-1 Exon1_MND-CD19CAR construct
  source 1..7609: mol_type = other DNA
cagctgcgcgctcgctcgctcactgaggccgcccgggcaaagcccgggcgtcgggcgacctttggtcgcccggcctcagtgagcgagcgagcgcgcagagagggagtggccaactccatcactaggggttccttgtagttaatgattaacccgccatgctacttatctacgtaaggctgttgcaggcatcacacggtggaaagatctggaactgtggccatggtgtgaggccatccacaaggtggaagctttgagggggagccgattagccatggacagttgtcattcagtagggtcacctgtgccccagcgaagggggatgggccgggaaggcagaggccaggcacctgcccccagcaggggcagaggctgtgggcagccgggaggctcccagaggctccgacagaatgggagtggggttgagcccacccctcactgcagcccaggaacctgagcccagagggggccacccaccttccccaggcagggaggcccggcccccagggagatgggggggatgggggaggagaagggcctgcccccacccggcagcctcaggaggggcagctcgggcgggatatggaaagaggccacagcagtgagcagagacacagaggaggaaggggccctgagctggggagacccccacggggtagggcgtgggggccacgggcccacctcctccccatctcctctgtctccctgtctctgtctctctctccctcccccaccctctccccagtcctaccccctcctcacccctcctcccccagcactgcctctgtcactctcgcccacgtggatgtggaggaagagggggcgggagcaaggggcgggcaccctcccttcaacctgacctgggacagtttcccttccgctcacctccgcctgagcagtggagaaggcggcactctggtggggctgctccaacgcgtgatccatcgattagtccaatttgttaaagacaggatatcagtggtccaggctctagttttgactcaacaatatcaccagctgaagcctatagagtacgagccatagatagaataaaagattttatttagtctccagaaaaaggggggaatgaaagaccccacctgtaggtttggcaagctaggatcaaggttaggaacagagagacagcagaatatgggccaaacaggatatctgtggtaagcagttcctgccccggctcagggccaagaacagttggaacagcagaatatgggccaaacaggatatctgtggtaagcagttcctgccccggctcagggccaagaacagatggtccccagatgcggtcccgccctcagcagtttctagagaaccatcagatgtttccagggtgccccaaggacctgaaatgaccctgtgccttatttgaactaaccaatcagttcgcttctcgcttctgttcgcgcgcttctgctccccgagctcaataaaagagcccacaacccctcactcggcgcgacgcgtcatagccaccatggccttaccagtgaccgccttgctcctgccgctggccttgctgctccacgccgccaggccggacatccagatgacacagactacatcctccctgtctgcctctctgggagacagagtcaccatcagttgcagggcaagtcaggacattagtaaatatttaaattggtatcagcagaaaccagatggaactgttaaactcctgatctaccatacatcaagattacactcaggagtcccatcaaggttcagtggcagtgggtctggaacagattattctctcaccattagcaacctggagcaagaagatattgccacttacttttgccaacagggtaatacgcttccgtacacgttcggaggggggaccaagctggagatcacaggtggcggtggctccggcggtggtgggtctggtggcggcggaagcgaggtgaaactgcaggagtcaggacctggcctggtggcgccctcacagagcctgtccgtcacatgcactgtctcaggggtctcattacccgactatggtgtaagctggattcgccagcctccacgaaagggtctggagtggctgggagtaatatggggtagtgaaaccacatactataattcagctctcaaatccagactgaccatcatcaaggacaactccaagagccaagttttcttaaaaatgaacagtctgcaaactgatgacacagccatttactactgtgccaaacattattactacggtggtagctatgctatggactactggggtcaaggaacctcggtcaccgtctcctcaaccacgacgccagcgccgcgaccaccaacaccggcgcccaccatcgcgtcgcagcccctgtccctgcgcccagaggcgtgccggccagcggcggggggcgcagtgcacacgagggggctggacttcgcctgtgatatctacatctgggcgcccttggccgggacttgtggggtccttctcctgtcactggtgatcaccctttactgcaaacggggcagaaagaaactcctgtatatattcaaacaaccatttatgagaccagtacaaactactcaagaggaagatggctgtagctgccgatttccagaagaagaagaaggaggatgtgaactgagagtgaagttcagcaggagcgcagacgcccccgcgtaccagcagggccagaaccagctctataacgagctcaatctaggacgaagagaggagtacgatgttttggacaagagacgtggccgggaccctgagatggggggaaagccgagaaggaagaaccctcaggaaggcctgtacaatgaactgcagaaagataagatggcggaggcctacagtgagattgggatgaaaggcgagcgccggaggggcaaggggcacgatggcctttaccagggtctcagtacagccaccaaggacacctacgacgcccttcacatgcaggccctgccccctcgctaagcggccgcgctttatttgtgaaatttgtgatgctattgctttatttgtaaccattataagctgcaataaacaagttaacaacaacaattgcattcattttatgtttcaggttcagggggagatgtgggaggttttttaaagctcaccggttctgggcggtgctacaactgggctggcggccaggatggttcttaggtaggtggggtcggcggtcaggtgtcccagagccaggggtctggagggaccttccaccctcagtccctggcaggtcggggggtgctgaggcgggcctggccctggcagcccaggggtcccggagcgaggggtctggagggacctttcactctcagtccctggcaggtcggggggtgctgtggcaggcccagccttggcccccagctctgccccttaccctgagctgtgtggctttgggcagctcgaactcctgggttcctctctgggccccaactcctcccctggcccaagtcccctctttgctcctgggcaggcaggacctctgtcccctctcagccggtccttggggctgcgtgtttctgtagaatgacgggtcaggctggccagaaccccaaaccttggccgtggggagtctgcgtggcggctctgccttgcccaggcatccttggtcctcactcgagttttcctaaggatgggatgagccccatgtgggactaaccttggctttacgacgtcaaagtttagatgagctggtgatatttttctcattatatccaaagtgtacctgttcgagtgaggacagttcttctgtctccaggatccctcctgggtggggattgtgcccgcctgggtctctgcccagattccagggctctccccgagccctgttcagaccatccgtgggggaggccttggcctcactcttacgtagataagtagcatggcgggttaatcattaactacaaggaacccctagtgatggagttggccactccctctctgcgcgctcgctcgctcactgaggccgggcgaccaaaggtcgcccgacgcccgggctttgcccgggcggcctcagtgagcgagcgagcgcgccagctggcgtaatagcgaagaggcccgcaccgatcgcccttcccaacagttgcgcagcctgaatggcgaatggcgattccgttgcaatggctggcggtaatattgttctggatattaccagcaaggccgatagtttgagttcttctactcaggcaagtgatgttattactaatcaaagaagtattgcgacaacggttaatttgcgtgatggacagactcttttactcggtggcctcactgattataaaaacacttctcaggattctggcgtaccgttcctgtctaaaatccctttaatcggcctcctgtttagctcccgctctgattctaacgaggaaagcacgttatacgtgctcgtcaaagcaaccatagtacgcgccctgtagcggcgcattaagcgcggcgggtgtggtggttacgcgcagcgtgaccgctacacttgccagcgccctagcgcccgctcctttcgctttcttcccttcctttctcgccacgttcgccggctttccccgtcaagctctaaatcgggggctccctttagggttccgatttagtgctttacggcacctcgaccccaaaaaacttgattagggtgatggttcacgtagtgggccatcgccctgatagacggtttttcgccctttgacgttggagtccacgttctttaatagtggactcttgttccaaactggaacaacactcaaccctatctcggtctattcttttgatttataagggattttgccgatttcggcctattggttaaaaaatgagctgatttaacaaaaatttaacgcgaattttaacaaaatattaacgtttacaatttaaatatttgcttatacaatcttcctgtttttggggcttttctgattatcaaccggggtacatatgattgacatgctagttttacgattaccgttcatcgattctcttgtttgctccagactctcaggcaatgacctgatagcctttgtagagacctctcaaaaatagctaccctctccggcatgaatttatcagctagaacggttgaatatcatattgatggtgatttgactgtctccggcctttctcacccgtttgaatctttacctacacattactcaggcattgcatttaaaatatatgagggttctaaaaatttttatccttgcgttgaaataaaggcttctcccgcaaaagtattacagggtcataatgtttttggtacaaccgatttagctttatgctctgaggctttattgcttaattttgctaattctttgccttgcctgtatgatttattggatgttggaatcgcctgatgcggtattttctccttacgcatctgtgcggtatttcacaccgcatatggtgcactctcagtacaatctgctctgatgccgcatagttaagccagccccgacacccgccaacacccgctgacgcgccctgacgggcttgtctgctcccggcatccgcttacagacaagctgtgaccgtctccgggagctgcatgtgtcagaggttttcaccgtcatcaccgaaacgcgcgagacgaaagggcctcgtgatacgcctatttttataggttaatgtcatgataataatggtttcttagacgtcaggtggcacttttcggggaaatgtgcgcggaacccctatttgtttatttttctaaatacattcaaatatgtatccgctcatgagacaataaccctgataaatgcttcaataatattgaaaaaggaagagtatgagtattcaacatttccgtgtcgcccttattcccttttttgcggcattttgccttcctgtttttgctcacccagaaacgctggtgaaagtaaaagatgctgaagatcagttgggtgcacgagtgggttacatcgaactggatctcaacagcggtaagatccttgagagttttcgccccgaagaacgttttccaatgatgagcacttttaaagttctgctatgtggcgcggtattatcccgtattgacgccgggcaagagcaactcggtcgccgcatacactattctcagaatgacttggttgagtactcaccagtcacagaaaagcatcttacggatggcatgacagtaagagaattatgcagtgctgccataaccatgagtgataacactgcggccaacttacttctgacaacgatcggaggaccgaaggagctaaccgcttttttgcacaacatgggggatcatgtaactcgccttgatcgttgggaaccggagctgaatgaagccataccaaacgacgagcgtgacaccacgatgcctgtagcaatggcaacaacgttgcgcaaactattaactggcgaactacttactctagcttcccggcaacaattaatagactggatggaggcggataaagttgcaggaccacttctgcgctcggcccttccggctggctggtttattgctgataaatctggagccggtgagcgtgggtctcgcggtatcattgcagcactggggccagatggtaagccctcccgtatcgtagttatctacacgacggggagtcaggcaactatggatgaacgaaatagacagatcgctgagataggtgcctcactgattaagcattggtaactgtcagaccaagtttactcatatatactttagattgatttaaaacttcatttttaatttaaaaggatctaggtgaagatcctttttgataatctcatgaccaaaatcccttaacgtgagttttcgttccactgagcgtcagaccccgtagaaaagatcaaaggatcttcttgagatcctttttttctgcgcgtaatctgctgcttgcaaacaaaaaaaccaccgctaccagcggtggtttgtttgccggatcaagagctaccaactctttttccgaaggtaactggcttcagcagagcgcagataccaaatactgtccttctagtgtagccgtagttaggccaccacttcaagaactctgtagcaccgcctacatacctcgctctgctaatcctgttaccagtggctgctgccagtggcgataagtcgtgtcttaccgggttggactcaagacgatagttaccggataaggcgcagcggtcgggctgaacggggggttcgtgcacacagcccagcttggagcgaacgacctacaccgaactgagatacctacagcgtgagctatgagaaagcgccacgcttcccgaagggagaaaggcggacaggtatccggtaagcggcagggtcggaacaggagagcgcacgagggagcttccagggggaaacgcctggtatctttatagtcctgtcgggtttcgccacctctgacttgagcgtcgatttttgtgatgctcgtcaggggggcggagcctatggaaaaacgccagcaacgcggcctttttacggttcctggccttttgctggccttttgctcacatgttctttcctgcgttatcccctgattctgtggataaccgtattaccgcctttgagtgagctgataccgctcgccgcagccgaacgaccgagcgcagcgagtcagtgagcgaggaagcggaagagcgcccaatacgcaaaccgcctctccccgcgcgttggccgattcattaatg

SEQ ID NO: 57 - DNA, 7492 bp, synthetic construct
  misc_feature 1..7492: note = Synthesized rAAV PD-1 Exon1_MND-BCMACAR construct
  source 1..7492: mol_type = other DNA
cagctgcgcgctcgctcgctcactgaggccgcccgggcaaagcccgggcgtcgggcgacctttggtcgcccggcctcagtgagcgagcgagcgcgcagagagggagtggccaactccatcactaggggttccttgtagttaatgattaacccgccatgctacttatctacgtaaggctgttgcaggcatcacacggtggaaagatctggaactgtggccatggtgtgaggccatccacaaggtggaagctttgagggggagccgattagccatggacagttgtcattcagtagggtcacctgtgccccagcgaagggggatgggccgggaaggcagaggccaggcacctgcccccagcaggggcagaggctgtgggcagccgggaggctcccagaggctccgacagaatgggagtggggttgagcccacccctcactgcagcccaggaacctgagcccagagggggccacccaccttccccaggcagggaggcccggcccccagggagatgggggggatgggggaggagaagggcctgcccccacccggcagcctcaggaggggcagctcgggcgggatatggaaagaggccacagcagtgagcagagacacagaggaggaaggggccctgagctggggagacccccacggggtagggcgtgggggccacgggcccacctcctccccatctcctctgtctccctgtctctgtctctctctccctcccccaccctctccccagtcctaccccctcctcacccctcctcccccagcactgcctctgtcactctcgcccacgtggatgtggaggaagagggggcgggagcaaggggcgggcaccctcccttcaacctgacctgggacagtttcccttccgctcacctccgcctgagcagtggagaaggcggcactctggtggggctgctccaacgcgtaatgaaagaccccacctgtaggtttggcaagctaggatcaaggttaggaacagagagacagcagaatatgggccaaacaggatatctgtggtaagcagttcctgccccggctcagggccaagaacagttggaacagcagaatatgggccaaacaggatatctgtggtaagcagttcctgccccggctcagggccaagaacagatggtccccagatgcggtcccgccctcagcagtttctagagaaccatcagatgtttccagggtgccccaaggacctgaaatgaccctgtgccttatttgaactaaccaatcagttcgcttctcgcttctgttcgcgcgcttctgctccccgagctcaataaaagagcccacaacccctcactcggcgcgattcacctgacgcgtctacgccaccatggcactccccgtcaccgcccttctcttgcccctcgccctgctgctgcatgctgccaggcccgacattgtgctcactcagtcacctcccagcctggccatgagcctgggaaaaagggccaccatctcctgtagagccagtgagtccgtcacaatcttggggagccatcttattcactggtatcagcagaagcccgggcagcctccaacccttcttattcagctcgcgtcaaacgtccagacgggtgtacctgccagattttctggtagcgggtcccgcactgattttacactgaccatagatccagtggaagaagacgatgtggccgtgtattattgtctgcagagcagaacgattcctcgcacatttggtgggggtactaagctggagattaagggaagcacgtccggctcagggaagccgggctccggcgagggaagcacgaaggggcaaattcagctggtccagagcggacctgagctgaaaaaacccggcgagactgttaagatcagttgtaaagcatctggctataccttcaccgactacagcataaattgggtgaaacgggcccctggaaagggcctcaaatggatgggttggatcaataccgaaactagggagcctgcttatgcatatgacttccgcgggagattcgccttttcactcgagacatctgcctctactgcttacctccaaataaacaacctcaagtatgaagatacagccacttacttttgcgccctcgactatagttacgccatggactactggggacagggaacctccgttaccgtcagttccgcggccgcaaccacaacacctgctccaaggccccccacacccgctccaactatagccagccaaccattgagcctcagacctgaagcttgcaggcccgcagcaggaggcgccgtccatacgcgaggcctggacttcgcgtgtgatatttatatttgggcccctttggccggaacatgtggggtgttgcttctctcccttgtgatcactctgtattgtaagcgcgggagaaagaagctcctgtacatcttcaagcagccttttatgcgacctgtgcaaaccactcaggaagaagatgggtgttcatgccgcttccccgaggaggaagaaggagggtgtgaactgagggtgaaattttctagaagcgccgatgctcccgcatatcagcagggtcagaatcagctctacaatgaattgaatctcggcaggcgagaagagtacgatgttctggacaagagacggggcagggatcccgagatggggggaaagccccggagaaaaaatcctcaggaggggttgtacaatgagctgcagaaggacaagatggctgaagcctatagcgagatcggaatgaaaggcgaaagacgcagaggcaaggggcatgacggtctgtaccagggtctctctacagccaccaaggacacttatgatgcgttgcatatgcaagccttgccaccccgctaagcggccgcgctttatttgtgaaatttgtgatgctattgctttatttgtaaccattataagctgcaataaacaagttaacaacaacaattgcattcattttatgtttcaggttcagggggagatgtgggaggttttttaaagctcaccggttctgggcggtgctacaactgggctggcggccaggatggttcttaggtaggtggggtcggcggtcaggtgtcccagagccaggggtctggagggaccttccaccctcagtccctggcaggtcggggggtgctgaggcgggcctggccctggcagcccaggggtcccggagcgaggggtctggagggacctttcactctcagtccctggcaggtcggggggtgctgtggcaggcccagccttggcccccagctctgccccttaccctgagctgtgtggctttgggcagctcgaactcctgggttcctctctgggccccaactcctcccctggcccaagtcccctctttgctcctgggcaggcaggacctctgtcccctctcagccggtccttggggctgcgtgtttctgtagaatgacgggtcaggctggccagaaccccaaaccttggccgtggggagtctgcgtggcggctctgccttgcccaggcatccttggtcctcactcgagttttcctaaggatgggatgagccccatgtgggactaaccttggctttacgacgtcaaagtttagatgagctggtgatatttttctcattatatccaaagtgtacctgttcgagtgaggacagttcttctgtctccaggatccctcctgggtggggattgtgcccgcctgggtctctgcccagattccagggctctccccgagccctgttcagaccatccgtgggggaggccttggcctcactcttacgtagataagtagcatggcgggttaatcattaactacaaggaacccctagtgatggagttggccactccctctctgcgcgctcgctcgctcactgaggccgggcgaccaaaggtcgcccgacgcccgggctttgcccgggcggcctcagtgagcgagcgagcgcgccagctggcgtaatagcgaagaggcccgcaccgatcgcccttcccaacagttgcgcagcctgaatggcgaatggcgattccgttgcaatggctggcggtaatattgttctggatattaccagcaaggccgatagtttgagttcttctactcaggcaagtgatgttattactaatcaaagaagtattgcgacaacggttaatttgcgtgatggacagactcttttactcggtggcctcactgattataaaaacacttctcaggattctggcgtaccgttcctgtctaaaatccctttaatcggcctcctgtttagctcccgctctgattctaacgaggaaagcacgttatacgtgctcgtcaaagcaaccatagtacgcgccctgtagcggcgcattaagcgcggcgggtgtggtggttacgcgcagcgtgaccgctacacttgccagcgccctagcgcccgctcctttcgctttcttcccttcctttctcgccacgttcgccggctttccccgtcaagctctaaatcgggggctccctttagggttccgatttagtgctttacggcacctcgaccccaaaaaacttgattagggtgatggttcacgtagtgggccatcgccctgatagacggtttttcgccctttgacgttggagtccacgttctttaatagtggactcttgttccaaactggaacaacactcaaccctatctcggtctattcttttgatttataagggattttgccgatttcggcctattggttaaaaaatgagctgatttaacaaaaatttaacgcgaattttaacaaaatattaacgtttacaatttaaatatttgcttatacaatcttcctgtttttggggcttttctgattatcaaccggggtacatatgattgacatgctagttttacgattaccgttcatcgattctcttgtttgctccagactctcaggcaatgacctgatagcctttgtagagacctctcaaaaatagctaccctctccggcatgaatttatcagctagaacggttgaatatcatattgatggtgatttgactgtctccggcctttctcacccgtttgaatctttacctacacattactcaggcattgcatttaaaatatatgagggttctaaaaatttttatccttgcgttgaaataaaggcttctcccgcaaaagtattacagggtcataatgtttttggtacaaccgatttagctttatgctctgaggctttattgcttaattttgctaattctttgccttgcctgtatgatttattggatgttggaatcgcctgatgcggtattttctccttacgcatctgtgcggtatttcacaccgcatatggtgcactctcagtacaatctgctctgatgccgcatagttaagccagccccgacacccgccaacacccgctgacgcgccctgacgggcttgtctgctcccggcatccgcttacagacaagctgtgaccgtctccgggagctgcatgtgtcagaggttttcaccgtcatcaccgaaacgcgcgagacgaaagggcctcgtgatacgcctatttttataggttaatgtcatgataataatggtttcttagacgtcaggtggcacttttcggggaaatgtgcgcggaacccctatttgtttatttttctaaatacattcaaatatgtatccgctcatgagacaataaccctgataaatgcttcaataatattgaaaaaggaagagtatgagtattcaacatttccgtgtcgcccttattcccttttttgcggcattttgccttcctgtttttgctcacccagaaacgctggtgaaagtaaaagatgctgaagatcagttgggtgcacgagtgggttacatcgaactggatctcaacagcggtaagatccttgagagttttcgccccgaagaacgttttccaatgatgagcacttttaaagttctgctatgtggcgcggtattatcccgtattgacgccgggcaagagcaactcggtcgccgcatacactattctcagaatgacttggttgagtactcaccagtcacagaaaagcatcttacggatggcatgacagtaagagaattatgcagtgctgccataaccatgagtgataacactgcggccaacttacttctgacaacgatcggaggaccgaaggagctaaccgcttttttgcacaacatgggggatcatgtaactcgccttgatcgttgggaaccggagctgaatgaagccataccaaacgacgagcgtgacaccacgatgcctgtagcaatggcaacaacgttgcgcaaactattaactggcgaactacttactctagcttcccggcaacaattaatagactggatggaggcggataaagttgcaggaccacttctgcgctcggcccttccggctggctggtttattgctgataaatctggagccggtgagcgtgggtctcgcggtatcattgcagcactggggccagatggtaagccctcccgtatcgtagttatctacacgacggggagtcaggcaactatggatgaacgaaatagacagatcgctgagataggtgcctcactgattaagcattggtaactgtcagaccaagtttactcatatatactttagattgatttaaaacttcatttttaatttaaaaggatctaggtgaagatcctttttgataatctcatgaccaaaatcccttaacgtgagttttcgttccactgagcgtcagaccccgtagaaaagatcaaaggatcttcttgagatcctttttttctgcgcgtaatctgctgcttgcaaacaaaaaaaccaccgctaccagcggtggtttgtttgccggatcaagagctaccaactctttttccgaaggtaactggcttcagcagagcgcagataccaaatactgtccttctagtgtagccgtagttaggccaccacttcaagaactctgtagcaccgcctacatacctcgctctgctaatcctgttaccagtggctgctgccagtggcgataagtcgtgtcttaccgggttggactcaagacgatagttaccggataaggcgcagcggtcgggctgaacggggggttcgtgcacacagcccagcttggagcgaacgacctacaccgaactgagatacctacagcgtgagctatgagaaagcgccacgcttcccgaagggagaaaggcggacaggtatccggtaagcggcagggtcggaacaggagagcgcacgagggagcttccagggggaaacgcctggtatctttatagtcctgtcgggtttcgccacctctgacttgagcgtcgatttttgtgatgctcgtcaggggggcggagcctatggaaaaacgccagcaacgcggcctttttacggttcctggccttttgctggccttttgctcacatgttctttcctgcgttatcccctgattctgtggataaccgtattaccgcctttgagtgagctgataccgctcgccgcagccgaacgaccgagcgcagcgagtcagtgagcgaggaagcggaagagcgcccaatacgcaaaccgcctctccccgcgcgttggccgattcattaatg

SEQ ID NO: 58 - DNA, 6147 bp, synthetic construct
  misc_feature 1..6147: note = Synthesized rAAV PD-1 Exon1_ATG-mCherry construct
  source 1..6147: mol_type = other DNA
cagctgcgcgctcgctcgctcactgaggccgcccgggcaaagcccgggcgtcgggcgacctttggtcgcccggcctcagtgagcgagcgagcgcgcagagagggagtggccaactccatcactaggggttccttgtagttaatgattaacccgccatgctacttatctacgtaaggctgttgcaggcatcacacggtggaaagatctggaactgtggccatggtgtgaggccatccacaaggtggaagctttgagggggagccgattagccatggacagttgtcattcagtagggtcacctgtgccccagcgaagggggatgggccgggaaggcagaggccaggcacctgcccccagcaggggcagaggctgtgggcagccgggaggctcccagaggctccgacagaatgggagtggggttgagcccacccctcactgcagcccaggaacctgagcccagagggggccacccaccttccccaggcagggaggcccggcccccagggagatgggggggatgggggaggagaagggcctgcccccacccggcagcctcaggaggggcagctcgggcgggatatggaaagaggccacagcagtgagcagagacacagaggaggaaggggccctgagctggggagacccccacggggtagggcgtgggggccacgggcccacctcctccccatctcctctgtctccctgtctctgtctctctctccctcccccaccctctccccagtcctaccccctcctcacccctcctcccccagcactgcctctgtcactctcgcccacgtggatgtggaggaagagggggcgggagcaaggggcgggcaccctcccttcaacctgacctgggacagtttcccttccgctcacctccgcctgagcagtggagaaggcggcactctggtggggctgctccaggcatgcaggtgagcaagggcgaggaggataactccgccatcatcaaggagttcctgcgcttcaaggtgcacatggagggctccgtgaacggccacgagttcgagatcgagggcgagggcgagggccgcccctacgagggcacccagaccgccaagctgaaggtgaccaagggtggccccctgcccttcgcctgggacatcctgtcccctcagttcatgtacggctccaaggcctacgtgaagcaccccgccgacatccccgactacttgaagctgtccttccccgagggcttcaagtgggagcgcgtgatgaacttcgaggacggcggcgtggtgaccgtgacccaggactcctctctgcaggacggcgagttcatctacaaggtgaagctgcgcggcaccaacttcccctccgacggccccgtaatgcagaagaagaccatgggctgggaggcctcctccgagcggatgtaccccgaggacggcgccctgaagggcgagatcaagcagaggctgaagctgaaggacggcggccactacgacgctgaggtcaagaccacctacaaggccaagaagcccgtgcagctgcccggcgcctacaacgtcaacatcaagttggacatcacctcccacaacgaggactacaccatcgtggaacagtacgaacgcgccgagggccgccactccaccggcggcatggacgagctgtacaagtgatgaaagctttgctttatttgtgaaatttgtgatgctatgctttatttgtaaccattataagctgcaataaacaagtttaacaacaacaattgcattcattttatgtttcaggttcagggggaggtgtgggaggttttttaaagtaggtggggtcggcggtcaggtgtcccagagccaggggtctggagggaccttccaccctcagtccctggcaggtcggggggtgctgaggcgggcctggccctggcagcccaggggtcccggagcgaggggtctggagggacctttcactctcagtccctggcaggtcggggggtgctgtggcaggcccagccttggcccccagctctgccccttaccctgagctgtgtggctttgggcagctcgaactcctgggttcctctctgggccccaactcctcccctggcccaagtcccctctttgctcctgggcaggcaggacctctgtcccctctcagccggtccttggggctgcgtgtttctgtagaatgacgggtcaggctggccagaaccccaaaccttggccgtggggagtctgcgtggcggctctgccttgcccaggcatccttggtcctcactcgagttttcctaaggatgggatgagccccatgtgggactaaccttggctttacgacgtcaaagtttagatgagctggtgatatttttctcattatatccaaagtgtacctgttcgagtgaggacagttcttctgtctccaggatacgtagataagtagcatggcgggttaatcattaactacaaggaacccctagtgatggagttggccactccctctctgcgcgctcgctcgctcactgaggccgggcgaccaaaggtcgcccgacgcccgggctttgcccgggcggcctcagtgagcgagcgagcgcgccagctggcgtaatagcgaagaggcccgcaccgatcgcccttcccaacagttgcgcagcctgaatggcgaatggcgattccgttgcaatggctggcggtaatattgttctggatattaccagcaaggccgatagtttgagttcttctactcaggcaagtgatgttattactaatcaaagaagtattgcgacaacggttaatttgcgtgatggacagactcttttactcggtggcctcactgattataaaaacacttctcaggattctggcgtaccgttcctgtctaaaatccctttaatcggcctcctgtttagctcccgctctgattctaacgaggaaagcacgttatacgtgctcgtcaaagcaaccatagtacgcgccctgtagcggcgcattaagcgcggcgggtgtggtggttacgcgcagcgtgaccgctacacttgccagcgccctagcgcccgctcctttcgctttcttcccttcctttctcgccacgttcgccggctttccccgtcaagctctaaatcgggggctccctttagggttccgatttagtgctttacggcacctcgaccccaaaaaacttgattagggtgatggttcacgtagtgggccatcgccctgatagacggtttttcgccctttgacgttggagtccacgttctttaatagtggactcttgttccaaactggaacaacactcaaccctatctcggtctattcttttgatttataagggattttgccgatttcggcctattggttaaaaaatgagctgatttaacaaaaatttaacgcgaattttaacaaaatattaacgtttacaatttaaatatttgcttatacaatcttcctgtttttggggcttttctgattatcaaccggggtacatatgattgacatgctagttttacgattaccgttcatcgattctcttgtttgctccagactctcaggcaatgacctgatagcctttgtagagacctctcaaaaatagctaccctctccggcatgaatttatcagctagaacggttgaatatcatattgatggtgatttgactgtctccggcctttctcacccgtttgaatctttacctacacattactcaggcattgcatttaaaatatatgagggttctaaaaatttttatccttgcgttgaaataaaggcttctcccgcaaaagtattacagggtcataatgtttttggtacaaccgatttagctttatgctctgaggctttattgcttaattttgctaattctttgccttgcctgtatgatttattggatgttggaatcgcctgatgcggtattttctccttacgcatctgtgcggtatttcacaccgcatatggtgcactctcagtacaatctgctctgatgccgcatagttaagccagccccgacacccgccaacacccgctgacgcgccctgacgggcttgtctgctcccggcatccgcttacagacaagctgtgaccgtctccgggagctgcatgtgtcagaggttttcaccgtcatcaccgaaacgcgcgagacgaaagggcctcgtgatacgcctatttttataggttaatgtcatgataataatggtttcttagacgtcaggtggcacttttcggggaaatgtgcgcggaacccctatttgtttatttttctaaatacattcaaatatgtatccgctcatgagacaataaccctgataaatgcttcaataatattgaaaaaggaagagtatgagtattcaacatttccgtgtcgcccttattcccttttttgcggcattttgccttcctgtttttgctcacccagaaacgctggtgaaagtaaaagatgctgaagatcagttgggtgcacgagtgggttacatcgaactggatctcaacagcggtaagatccttgagagttttcgccccgaagaacgttttccaatgatgagcacttttaaagttctgctatgtggcgcggtattatcccgtattgacgccgggcaagagcaactcggtcgccgcatacactattctcagaatgacttggttgagtactcaccagtcacagaaaagcatcttacggatggcatgacagtaagagaattatgcagtgctgccataaccatgagtgataacactgcggccaacttacttctgacaacgatcggaggaccgaaggagctaaccgcttttttgcacaacatgggggatcatgtaactcgccttgatcgttgggaaccggagctgaatgaagccataccaaacgacgagcgtgacaccacgatgcctgtagcaatggcaacaacgttgcgcaaactattaactggcgaactacttactctagcttcccggcaacaattaatagactggatggaggcggataaagttgcaggaccacttctgcgctcggcccttccggctggctggtttattgctgataaatctggagccggtgagcgtgggtctcgcggtatcattgcagcactggggccagatggtaagccctcccgtatcgtagttatctacacgacggggagtcaggcaactatggatgaacgaaatagacagatcgctgagataggtgcctcactgattaagcattggtaactgtcagaccaagtttactcatatatactttagattgatttaaaacttcatttttaatttaaaaggatctaggtgaagatcctttttgataatctcatgaccaaaatcccttaacgtgagttttcgttccactgagcgtcagaccccgtagaaaagatcaaaggatcttcttgagatcctttttttctgcgcgtaatctgctgcttgcaaacaaaaaaaccaccgctaccagcggtggtttgtttgccggatcaagagctaccaactctttttccgaaggtaactggcttcagcagagcgcagataccaaatactgtccttctagtgtagccgtagttaggccaccacttcaagaactctgtagcaccgcctacatacctcgctctgctaatcctgttaccagtggctgctgccagtggcgataagtcgtgtcttaccgggttggactcaagacgatagttaccggataaggcgcagcggtcgggctgaacggggggttcgtgcacacagcccagcttggagcgaacgacctacaccgaactgagatacctacagcgtgagctatgagaaagcgccacgcttcccgaagggagaaaggcggacaggtatccggtaagcggcagggtcggaacaggagagcgcacgagggagcttccagggggaaacgcctggtatctttatagtcctgtcgggtttcgccacctctgacttgagcgtcgatttttgtgatgctcgtcaggggggcggagcctatggaaaaacgccagcaacgcggcctttttacggttcctggccttttgctggccttttgctcacatgttctttcctgcgttatcccctgattctgtggataaccgtattaccgcctttgagtgagctgataccgctcgccgcagccgaacgaccgagcgcagcgagtcagtgagcgaggaagcggaagagcgcccaatacgcaaaccgcctctccccgcgcgttggccgattcattaatg

SEQ ID NO: 59 - protein, 232 aa, synthetic construct
  REGION 1..232: note = Made in Lab
MQIPQAPWPVVWAVLQLGWRPGWFLDSPDRPWNPPTFSPALLVVTEGDNATFTCSFSNTSESFVLNWYRMSPSNQTDKLAAFPEDRSQPGQDCRFRVTQLPNGRDFHMSVVRARRNDSGTYLCGAISLAPKAQIKESLRAELRVTERRAEVPTAHPSPSPRPAGQFQTLVVGVVGGLLGSLVLLVWVLAVIRSKRSRLLHSDYMNMTPRRPGPTRKHYQPYAPPRDFAAYRS

SEQ ID NO: 60 - protein, 303 aa, synthetic construct; identical to SEQ ID NO: 6
  REGION 1..303: note = Synthesized I-OnuI variant PD-1.ile3.exon1_RD2_B1G2
  MOD_RES 1..4: note = Any amino acid or absent
  MOD_RES 302..303: note = Any amino acid or absent

SEQ ID NO: 61 - protein, 303 aa, synthetic construct
  REGION 1..303: note = Synthesized I-OnuI variant PD-1.ile3.exon1_RD3_B1G2C4
  MOD_RES 1..4: note = Any amino acid or absent
  MOD_RES 302..303: note = Any amino acid or absent
XXXXSRRESINPWILTGFADAEGSFGLSILNRNRGTARYHTRLSFTIMLHNKDKSILENIQSTWKVGSILNNGDHYVSLVVYRFEDLKVIIDHFEKYPLITQKLGDYKLFKQAFSVMENKEHLKENGIKELVRIKAKMNWGLNDELKKAFPENISKERPLINKNIPNFKWLAGFTSGDGSFFVRLRKSNVNARVRVQLVFEISQHIRDKNLMNSLITYLGCGHIYEGNKSERSWLQFRVEKFSDINDKIIPVFQENTLIGVKLEDFEDWCKVAKLIEEKKHLTESGLDEIKKIKLNMNKGRXX

SEQ ID NO: 62 - protein, 303 aa, synthetic construct
  REGION 1..303: note = Synthesized I-OnuI variant PD-1.ile3.exon1_RD3_B1 G2C11
  MOD_RES 1..4: note = Any amino acid or absent
  MOD_RES 302..303: note = Any amino acid or absent
XXXXSRRESINPWILTGFADAEGSFGLSILNRNRGTGRYHTRLSFTIMLHNKDKSILENIQSTWKVGSITNNGDHYVSLVVYRFEDLKVIIDHFEKYPLITQKLGDYKLFKQAFSVMENKEHLKENGIKELVRIKAKMNWGLNDELKKAFPENISKERPLINKNIPNFKWLAGFTSGDGSFFVRLRKSNVNARVRVQLVFEISQHIRDKNLMNSLITYLGCGHIYEGNKSERSWLQFRVEKFSDINDKIIPVFQENTLIGVKLEDFEDWCKVAKLIEEKKHLTESGLDEIKKIKLNMNKGRXX

SEQ ID NO: 63 - protein, 303 aa, synthetic construct
  REGION 1..303: note = Synthesized I-OnuI variant PD-1.ile3.exon1_RD3_B1 G2C5
  MOD_RES 1..4: note = Any amino acid or absent
  MOD_RES 302..303: note = Any amino acid or absent
XXXXSRRESINPWILTGFADAEGSFGLSILNRNRGTARYHTRLSFTIMLHNKDKSILENIQSTWKVGSIYNNGDHYVSLEVFRFEDLKVIIDHFEKYPLITQKLGDYKLFKQAFSVMENKEHLKENGIKELVRIKAKMNWGLNDELKKAFPENISKERPLINKNIPNFKWLAGFTSGDGSFFVRLRKSNVNARVRVQLVFEISQHIRDKNLMNSLITYLGCGHIYEGNKSERSWLQFRVEKFSDINDKIIPVFQENTLIGVKLEDFEDWCKVAKLIEEKKHLTESGLDEIKKIKLNMNKGRXX

SEQ ID NO: 64 - protein, 943 aa, synthetic construct
  REGION 1..943: note = Synthesized megaTAL PD-1.ile3.exon1_RD1_B1G2 construct
MGSAPPKKKRKVVDLRTLGYSQQQQEKIKPKVRSTVAQHHEALVGHGFTHAHIVALSQHPAALGTVAVTYQHIITALPEATHEDIVGVGKQWSGARALEALLTDAGELRGPPLQLDTGQLVKIAKRGGVTAMEAVHASRNALTGAPLNLTPDQVVAIASNNGGKQALETVQRLLPVLCQDHGLTPDQVVAIASNNGGKQALETVQRLLPVLCQDHGLTPDQVVAIASNGGGKQALETVQRLLPVLCQDHGLTPDQVVAIASNNGGKQALETVQRLLPVLCQDHGLTPDQVVAIASNNGGKQALETVQRLLPVLCQDHGLTPDQVVAIASNNGGKQALETVQRLLPVLCQDHGLTPDQVVAIASNNGGKQALETVQRLLPVLCQDHGLTPDQVVAIASHDGGKQALETVQRLLPVLCQDHGLTPDQVVAIASNGGGKQALETVQRLLPVLCQDHGLTPDQVVAIASNNGGKQALETVQRLLPVLCQDHGLTPDQVVAIASHDGGKQALETVQRLLPVLCQDHGLTPDQVVAIASNGGGKQALETVQRLLPVLCQDHGLTPDQVVAIASHDGGKQALESIVAQLSRPDPALAALTNDHLVALACLGGRPAMDAVKKGLPHAPELIRRVNRRIGERTSHRVAISRVGGSSRRESINPWILTGFADAEGSFGLSILNRNRGTARYHTRLSFTIMLHNKDKSILENIQSTWKVGIITNNGDHYVTLRVTRFEDLKVIIDHFEKYPLVTQKLGDYKLFKQAFSVMENKEHLKENGIKELVRIKAKMNWGLNDELKKAFPENISKERPLINKNIPNFKWLAGFTSGDGSFFVRLRKSNVNARVRVQLVFEISQHIRDKNLMNSLITYLGCGHIYEGNKSERSWLQFRVEKFSDINDKIIPVFQENTLIGVKLEDFEDWCKVAKLIEEKKHLTESGLDEIKKIKLNMNKGR

SEQ ID NO: 65 - RNA, 2832 nt, synthetic construct
  misc_feature 1..2832: note = Synthesized PD-1 Exon1 RD2_B1G2 megaTAL mRNA construct
  source 1..2832: mol_type = other RNA
atgggaagcgcgccacctaagaagaaacgcaaagtcgtggatctacgcacgctcggctacagtcagcagcagcaagagaagatcaaaccgaaggtgcgttcgacagtggcgcagcaccacgaggcactggtgggccatgggtttacacacgcgcacatcgttgcgctcagccaacacccggcagcgttagggaccgtcgctgtcacgtatcagcacataatcacggcgttgccagaggcgacacacgaagacatcgttggcgtcggcaaacagtggtccggcgcacgcgccctggaggccttgctcacggatgcgggggagttgagaggtccgccgttacagttggacacaggccaacttgtgaagattgcaaaacgtggcggcgtgaccgcaatggaggcagtgcatgcatcgcgcaatgcactgacgggtgcccccctgaacctaacccctgatcaggtagtcgctatagcttcaaacaacgggggcaagcaagcactggagaccgttcaacgactcctgccagtgctctgccaagaccacggacttacgccagatcaggtggttgctattgcctccaacaatggcgggaaacaagcgttggaaactgtgcagagactgttacctgtcttgtgtcaagaccacggcctcacgccagatcaggtggtagccatagcgtcgaatggaggtggtaagcaagcccttgaaacggtccagcgtcttctgccggtgttgtgccaggaccacggactaacgccggatcaggtcgtagccattgcttcaaataacggcggcaaacaggcgctagagacagtccagcgcctcttgcctgtgttatgccaggatcacggcttaaccccagaccaagttgtggctattgcatctaacaatggtggcaaacaagccttggagacagtgcaacgattactgcctgtcttatgtcaggatcatggcctgacgcccgatcaggtagtggcaatcgcatctaataatggaggtaagcaagcactggagactgtccagagattgttacccgtactatgtcaagatcatggtttgacgcctgatcaggttgttgcgatagccagcaacaacggagggaaacaggctcttgaaaccgtacagcgacttctcccagtcttgtgccaagatcacgggcttactcctgatcaagtcgtagctatcgccagccacgacggtgggaaacaggccctggaaaccgtacaacgtctcctcccagtactttgtcaagaccacgggttgactccggatcaagtcgtcgcgatcgcgagcaatggaggggggaagcaggcgctggaaactgttcagagactgctgcctgtactttgtcaggaccatggtctgacacctgaccaagttgtggcgatagccagtaacaatgggggaaaacaggcactagagacggttcaaaggttgttgcccgttctgtgccaggaccacggcttgacaccggatcaggtggtagctatcgcttcacacgatggcggaaaacaggctttagaaacagtccaaagacttctcccagtcctttgtcaggaccacggattgactccagatcaagtcgttgctattgcaagtaatggtggtggtaagcaagctttagaaaccgtacagaggcttttgccagtgctgtgccaggaccatggactgacccctgatcaagtggtagcaattgcatctcatgatggaggaaaacaagctctggaaagcattgtggcccagctgagccggcctgatccggcgttggccgcgttgaccaacgaccacctcgtcgccttggcctgcctcggcggacgtcctgccatggatgcagtgaaaaagggattgccgcacgcgccggaattgatcagaagagtcaatcgccgtattggcgaacgcacgtcccatcgcgttgcgatatctagagtgggaggaagctctcgcagagagtccatcaacccatggattctgactggtttcgctgatgccgaaggatcattcgggctaagcatcctcaacagaaacagaggtactgctagataccacactcgactgtcattcacaatcatgctgcacaacaaggacaaatcgattctggagaatatccagtcgacttggaaggtcggcataatcaccaacaacggcgaccactacgtcaccctgcgcgtcacccgtttcgaagatttgaaagtgattatcgaccacttcgagaaatatccgctggtaacacagaaattgggcgattacaagttgtttaaacaggcattcagcgtcatggagaacaaagaacatcttaaggagaatgggattaaggagctcgtacgaatcaaagctaagatgaattggggtctcaatgacgaattgaaaaaagcatttccagagaacattagcaaagagcgcccccttatcaataagaacattccgaatttcaaatggctggctggattcacatctggtgatggctccttcttcgtgcgcctaagaaagtctaatgttaatgctagagtacgtgtgcaactggtattcgagatctcacagcacatcagagacaagaacctgatgaattcattgataacatacctaggctgtggtcacatctacgagggaaacaaatctgagcgcagttggctccaattcagagtagaaaaattcagcgatatcaacgacaagatcattccggtattccaggaaaatactctgattggcgtcaaactcgaggactttgaagattggtgcaaggttgccaaattgatcgaagagaagaaacacctgaccgaatccggtttggatgagattaagaaaatcaagctgaacatgaacaaaggtcgttga

SEQ ID NO: 66 - RNA, 2832 nt, synthetic construct
  misc_feature 1..2832: note = Synthesized PD-1 Exon1 RD2_B1G2C4 megaTAL mRNA construct
  source 1..2832: mol_type = other RNA
atgggaagcgcgccacctaagaagaaacgcaaagtcgtggatctacgcacgctcggctacagtcagcagcagcaagagaagatcaaaccgaaggtgcgttcgacagtggcgcagcaccacgaggcactggtgggccatgggtttacacacgcgcacatcgttgcgctcagccaacacccggcagcgttagggaccgtcgctgtcacgtatcagcacataatcacggcgttgccagaggcgacacacgaagacatcgttggcgtcggcaaacagtggtccggcgcacgcgccctggaggccttgctcacggatgcgggggagttgagaggtccgccgttacagttggacacaggccaacttgtgaagattgcaaaacgtggcggcgtgaccgcaatggaggcagtgcatgcatcgcgcaatgcactgacgggtgcccccctgaacctaacccctgatcaggtagtcgctatagcttcaaacaacgggggcaagcaagcactggagaccgttcaacgactcctgccagtgctctgccaagaccacggacttacgccagatcaggtggttgctattgcctccaacaatggcgggaaacaagcgttggaaactgtgcagagactgttacctgtcttgtgtcaagaccacggcctcacgccagatcaggtggtagccatagcgtcgaatggaggtggtaagcaagcccttgaaacggtccagcgtcttctgccggtgttgtgccaggaccacggactaacgccggatcaggtcgtagccattgcttcaaataacggcggcaaacaggcgctagagacagtccagcgcctcttgcctgtgttatgccaggatcacggcttaaccccagaccaagttgtggctattgcatctaacaatggtggcaaacaagccttggagacagtgcaacgattactgcctgtcttatgtcaggatcatggcctgacgcccgatcaggtagtggcaatcgcatctaataatggaggtaagcaagcactggagactgtccagagattgttacccgtactatgtcaagatcatggtttgacgcctgatcaggttgttgcgatagccagcaacaacggagggaaacaggctcttgaaaccgtacagcgacttctcccagtcttgtgccaagatcacgggcttactcctgatcaagtcgtagctatcgccagccacgacggtgggaaacaggccctggaaaccgtacaacgtctcctcccagtactttgtcaagaccacgggttgactccggatcaagtcgtcgcgatcgcgagcaatggaggggggaagcaggcgctggaaactgttcagagactgctgcctgtactttgtcaggaccatggtctgacacctgaccaagttgtggcgatagccagtaacaatgggggaaaacaggcactagagacggttcaaaggttgttgcccgttctgtgccaggaccacggcttgacaccggatcaggtggtagctatcgcttcacacgatggcggaaaacaggctttagaaacagtccaaagacttctcccagtcctttgtcaggaccacggattgactccagatcaagtcgttgctattgcaagtaatggtggtggtaagcaagctttagaaaccgtacagaggcttttgccagtgctgtgccaggaccatggactgacccctgatcaagtggtagcaattgcatctcatgatggaggaaaacaagctctggaaagcattgtggcccagctgagccggcctgatccggcgttggccgcgttgaccaacgaccacctcgtcgccttggcctgcctcggcggacgtcctgccatggatgcagtgaaaaagggattgccgcacgcgccggaattgatcagaagagtcaatcgccgtattggcgaacgcacgtcccatcgcgttgcgatatctagagtgggaggaagctctcgcagagagtccatcaacccatggattctgactggtttcgctgatgccgaaggatcattcgggctaagcatcctcaacagaaacagaggtactgctagataccacactcgactgtcattcacaatcatgctgcacaacaaggacaaatcgattctggagaatatccagtcgacttggaaggtcggcagcatcctcaacaatggcgaccactacgtctcgctggtggtctaccgtttcgaagatttgaaagtgattatcgaccacttcgagaaatatccgctgataacacagaaattgggcgattacaagttgtttaaacaggcattcagcgtcatggagaacaaagaacatcttaaggagaatgggattaaggagctcgtacgaatcaaagctaagatgaattggggtctcaatgacgaattgaaaaaagcatttccagagaacattagcaaagagcgcccccttatcaataagaacattccgaatttcaaatggctggctggattcacatctggtgatggctccttcttcgtgcgcctaagaaagtctaatgttaatgctagagtacgtgtgcaactggtattcgagatctcacagcacatcagagacaagaacctgatgaattcattgataacatacctaggctgtggtcacatctacgagggaaacaaatctgagcgcagttggctccaattcagagtagaaaaattcagcgatatcaacgacaagatcattccggtattccaggaaaatactctgattggcgtcaaactcgaggactttgaagattggtgcaaggttgccaaattgatcgaagagaagaaacacctgaccgaatccggtttggatgagattaagaaaatcaagctgaacatgaacaaaggtcgttga

SEQ ID NO: 67 - RNA, 2832 nt, synthetic construct
  misc_feature 1..2832: note = Synthesized PD-1 Exon1 RD2_B1G2C11 megaTAL mRNA construct
  source 1..2832: mol_type = other RNA
atgggaagcgcgccacctaagaagaaacgcaaagtcgtggatctacgcacgctcggctacagtcagcagcagcaagagaagatcaaaccgaaggtgcgttcgacagtggcgcagcaccacgaggcactggtgggccatgggtttacacacgcgcacatcgttgcgctcagccaacacccggcagcgttagggaccgtcgctgtcacgtatcagcacataatcacggcgttgccagaggcgacacacgaagacatcgttggcgtcggcaaacagtggtccggcgcacgcgccctggaggccttgctcacggatgcgggggagttgagaggtccgccgttacagttggacacaggccaacttgtgaagattgcaaaacgtggcggcgtgaccgcaatggaggcagtgcatgcatcgcgcaatgcactgacgggtgcccccctgaacctaacccctgatcaggtagtcgctatagcttcaaacaacgggggcaagcaagcactggagaccgttcaacgactcctgccagtgctctgccaagaccacggacttacgccagatcaggtggttgctattgcctccaacaatggcgggaaacaagcgttggaaactgtgcagagactgttacctgtcttgtgtcaagaccacggcctcacgccagatcaggtggtagccatagcgtcgaatggaggtggtaagcaagcccttgaaacggtccagcgtcttctgccggtgttgtgccaggaccacggactaacgccggatcaggtcgtagccattgcttcaaataacggcggcaaacaggcgctagagacagtccagcgcctcttgcctgtgttatgccaggatcacggcttaaccccagaccaagttgtggctattgcatctaacaatggtggcaaacaagccttggagacagtgcaacgattactgcctgtcttatgtcaggatcatggcctgacgcccgatcaggtagtggcaatcgcatctaataatggaggtaagcaagcactggagactgtccagagattgttacccgtactatgtcaagatcatggtttgacgcctgatcaggttgttgcgatagccagcaacaacggagggaaacaggctcttgaaaccgtacagcgacttctcccagtcttgtgccaagatcacgggcttactcctgatcaagtcgtagctatcgccagccacgacggtgggaaacaggccctggaaaccgtacaacgtctcctcccagtactttgtcaagaccacgggttgactccggatcaagtcgtcgcgatcgcgagcaatggaggggggaagcaggcgctggaaactgttcagagactgctgcctgtactttgtcaggaccatggtctgacacctgaccaagttgtggcgatagccagtaacaatgggggaaaacaggcactagagacggttcaaaggttgttgcccgttctgtgccaggaccacggcttgacaccggatcaggtggtagctatcgcttcacacgatggcggaaaacaggctttagaaacagtccaaagacttctcccagtcctttgtcaggaccacggattgactccagatcaagtcgttgctattgcaagtaatggtggtggtaagcaagctttagaaaccgtacagaggcttttgccagtgctgtgccaggaccatggactgacccctgatcaagtggtagcaattgcatctcatgatggaggaaaacaagctctggaaagcattgtggcccagctgagccggcctgatccggcgttggccgcgttgaccaacgaccacctcgtcgccttggcctgcctcggcggacgtcctgccatggatgcagtgaaaaagggattgccgcacgcgccggaattgatcagaagagtcaatcgccgtattggcgaacgcacgtcccatcgcgttgcgatatctagagtgggaggaagctctcgcagagagtccatcaacccatggattctgactggtttcgctgatgccgaaggatcattcgggctaagcatcctcaacagaaacagaggtactggtagataccacactcgactgtcattcacaatcatgctgcacaacaaggacaaatcgattctggagaatatccagtcgacttggaaggtcggctcgatcacgaacaacggcgaccactacgtcagcctggtcgtctaccgtttcgaagatttgaaagtgattatcgaccacttcgagaaatatccgctgataacacagaaattgggcgattacaagttgtttaaacaggcattcagcgtcatggagaacaaagaacatcttaaggagaatgggattaaggagctcgtacgaatcaaagctaagatgaattggggtctcaatgacgaattgaaaaaagcatttccagagaacattagcaaagagcgcccccttatcaataagaacattccgaatttcaaatggctggctggattcacatctggtgatggctccttcttcgtgcgcctaagaaagtctaatgttaatgctagagtacgtgtgcaactggtattcgagatctcacagcacatcagagacaagaacctgatgaattcattgataacatacctaggctgtggtcacatctacgagggaaacaaatctgagcgcagttggctccaattcagagtagaaaaattcagcgatatcaacgacaagatcattccggtattccaggaaaatactctgattggcgtcaaactcgaggactttgaagattggtgcaaggttgccaaattgatcgaagagaagaaacacctgaccgaatccggtttggatgagattaagaaaatcaagctgaacatgaacaaaggtcgttga

SEQ ID NO: 68 - RNA, 2832 nt, synthetic construct
  misc_feature 1..2832: note = Synthesized PD-1 Exon1 RD2_B1G2C5 megaTAL mRNA construct
  source 1..2832: mol_type = other RNA
atgggaagcgcgccacctaagaagaaacgcaaagtcgtggatctacgcacgctcggctacagtcagcagcagcaagagaagatcaaaccgaaggtgcgttcgacagtggcgcagcaccacgaggcactggtgggccatgggtttacacacgcgcacatcgttgcgctcagccaacacccggcagcgttagggaccgtcgctgtcacgtatcagcacataatcacggcgttgccagaggcgacacacgaagacatcgttggcgtcggcaaacagtggtccggcgcacgcgccctggaggccttgctcacggatgcgggggagttgagaggtccgccgttacagttggacacaggccaacttgtgaagattgcaaaacgtggcggcgtgaccgcaatggaggcagtgcatgcatcgcgcaatgcactgacgggtgcccccctgaacctaacccctgatcaggtagtcgctatagcttcaaacaacgggggcaagcaagcactggagaccgttcaacgactcctgccagtgctctgccaagaccacggacttacgccagatcaggtggttgctattgcctccaacaatggcgggaaacaagcgttggaaactgtgcagagactgttacctgtcttgtgtcaagaccacggcctcacgccagatcaggtggtagccatagcgtcgaatggaggtggtaagcaagcccttgaaacggtccagcgtcttctgccggtgttgtgccaggaccacggactaacgccggatcaggtcgtagccattgcttcaaataacggcggcaaacaggcgctagagacagtccagcgcctcttgcctgtgttatgccaggatcacggcttaaccccagaccaagttgtggctattgcatctaacaatggtggcaaacaagccttggagacagtgcaacgattactgcctgtcttatgtcaggatcatggcctgacgcccgatcaggtagtggcaatcgcatctaataatggaggtaagcaagcactggagactgtccagagattgttacccgtactatgtcaagatcatggtttgacgcctgatcaggttgttgcgatagccagcaacaacggagggaaacaggctcttgaaaccgtacagcgacttctcccagtcttgtgccaagatcacgggcttactcctgatcaagtcgtagctatcgccagccacgacggtgggaaacaggccctggaaaccgtacaacgtctcctcccagtactttgtcaagaccacgggttgactccggatcaagtcgtcgcgatcgcgagcaatggaggggggaagcaggcgctggaaactgttcagagactgctgcctgtactttgtcaggaccatggtctgacacctgaccaagttgtggcgatagccagtaacaatgggggaaaacaggcactagagacggttcaaaggttgttgcccgttctgtgccaggaccacggcttgacaccggatcaggtggtagctatcgcttcacacgatggcggaaaacaggctttagaaacagtccaaagacttctcccagtcctttgtcaggaccacggattgactccagatcaagtcgttgctattgcaagtaatggtggtggtaagcaagctttagaaaccgtacagaggcttttgccagtgctgtgccaggaccatggactgacccctgatcaagtggtagcaattgcatctcatgatggaggaaaacaagctctggaaagcattgtggcccagctgagccggcctgatccggcgttggccgcgttgaccaacgaccacctcgtcgccttggcctgcctcggcggacgtcctgccatggatgcagtgaaaaagggattgccgcacgcgccggaattgatcagaagagtcaatcgccgtattggcgaacgcacgtcccatcgcgttgcgatatctagagtgggaggaagctctcgcagagagtccatcaacccatggattctgactggtttcgctgatgccgaaggatcattcgggctaagcatcctcaacagaaacagaggtactgctagataccacactcgactgtcattcacaatcatgctgcacaacaaggacaaatcgattctggagaatatccagtcgacttggaaggtcggctcgatctacaacaacggcgaccactacgtctcgctggaggtcttccgtttcgaagatttgaaagtgattatcgaccacttcgagaaatatccgctgataacacagaaattgggcgattacaagttgtttaaacaggcattcagcgtcatggagaacaaagaacatcttaaggagaatgggattaaggagctcgtacgaatcaaagctaagatgaattggggtctcaatgacgaattgaaaaaagcatttccagagaacattagcaaagagcgcccccttatcaataagaacattccgaatttcaaatggctggctggattcacatctggtgatggctccttcttcgtgcgcctaagaaagtctaatgttaatgctagagtacgtgtgcaactggtattcgagatctcacagcacatcagagacaagaacctgatgaattcattgataacatacctaggctgtggtcacatctacgagggaaacaaatctgagcgcagttggctccaattcagagtagaaaaattcagcgatatcaacgacaagatcattccggtattccaggaaaatactctgattggcgtcaaactcgaggactttgaagattggtgcaaggttgccaaattgatcgaagagaagaaacacctgaccgaatccggtttggatgagattaagaaaatcaagctgaacatgaacaaaggtcgttga

SEQ ID NO: 69 - skipped

SEQ ID NO: 70 - protein, 5 aa, synthetic construct
  REGION 1..5: note = Exemplary linker sequence
DGGGS

SEQ ID NO: 71 - protein, 5 aa, synthetic construct
  REGION 1..5: note = Exemplary linker sequence
TGEKP

SEQ ID NO: 72 - protein, 4 aa, synthetic construct
  REGION 1..4: note = Exemplary linker sequence
GGRR

SEQ ID NO: 73 - protein, 5 aa, synthetic construct
  REGION 1..5: note = Exemplary linker sequence
GGGGS

SEQ ID NO: 74 - protein, 14 aa, synthetic construct
  REGION 1..14: note = Exemplary linker sequence
EGKSSGSGSESKVD

SEQ ID NO: 75 - protein, 18 aa, synthetic construct
  REGION 1..18: note = Exemplary linker sequence
KESGSVSSEQLAQFRSLD

SEQ ID NO: 76 - protein, 8 aa, synthetic construct
  REGION 1..8: note = Exemplary linker sequence
GGRRGGGS

SEQ ID NO: 77 - protein, 9 aa, synthetic construct
  REGION 1..9: note = Exemplary linker sequence
LRQRDGERP

SEQ ID NO: 78 - protein, 12 aa, synthetic construct
  REGION 1..12: note = Exemplary linker sequence
LRQKDGGGSERP

SEQ ID NO: 79 - protein, 16 aa, synthetic construct
  REGION 1..16: note = Exemplary linker sequence
LRQKDGGGSGGGSERP

SEQ ID NO: 80 - skipped

SEQ ID NO: 81 - protein, 7 aa, synthetic construct
  REGION 1..7: note = Cleavage sequence by TEV protease
ENLYFQG

SEQ ID NO: 82 - protein, 7 aa, synthetic construct
  REGION 1..7: note = Cleavage sequence by TEV protease
ENLYFQS

SEQ ID NO: 83 - protein, 22 aa, synthetic construct
  REGION 1..22: note = Self-cleaving polypeptide comprising 2A site
GSGATNFSLLKQAGDVEENPGP

SEQ ID NO: 84 - protein, 19 aa, synthetic construct
  REGION 1..19: note = Self-cleaving polypeptide comprising 2A site
ATNFSLLKQAGDVEENPGP

SEQ ID NO: 85 - protein, 14 aa, synthetic construct
  REGION 1..14: note = Self-cleaving polypeptide comprising 2A site
LLKQAGDVEENPGP

SEQ ID NO: 86 - protein, 21 aa, synthetic construct
  REGION 1..21: note = Self-cleaving polypeptide comprising 2A site
GSGEGRGSLLTCGDVEENPGP

SEQ ID NO: 87 - protein, 18 aa, synthetic construct
  REGION 1..18: note = Self-cleaving polypeptide comprising 2A site
EGRGSLLTCGDVEENPGP

SEQ ID NO: 88 - protein, 13 aa, synthetic construct
  REGION 1..13: note = Self-cleaving polypeptide comprising 2A site
LLTCGDVEENPGP

SEQ ID NO: 89 - protein, 23 aa, synthetic construct
  REGION 1..23: note = Self-cleaving polypeptide comprising 2A site
GSGQCTNYALLKLAGDVESNPGP

SEQ ID NO: 90 - protein, 20 aa, synthetic construct
  REGION 1..20: note = Self-cleaving polypeptide comprising 2A site
QCTNYALLKLAGDVESNPGP

SEQ ID NO: 91 - protein, 14 aa, synthetic construct
  REGION 1..14: note = Self-cleaving polypeptide comprising 2A site
LLKLAGDVESNPGP

SEQ ID NO: 92 - protein, 25 aa, synthetic construct
  REGION 1..25: note = Self-cleaving polypeptide comprising 2A site
GSGVKQTLNFDLLKLAGDVESNPGP

SEQ ID NO: 93 - protein, 22 aa, synthetic construct
  REGION 1..22: note = Self-cleaving polypeptide comprising 2A site
VKQTLNFDLLKLAGDVESNPGP

SEQ ID NO: 94 - protein, 14 aa, synthetic construct
  REGION 1..14: note = Self-cleaving polypeptide comprising 2A site
LLKLAGDVESNPGP

SEQ ID NO: 95 - protein, 19 aa, synthetic construct
  REGION 1..19: note = Self-cleaving polypeptide comprising 2A site
LLNFDLLKLAGDVESNPGP

SEQ ID NO: 96 - protein, 19 aa, synthetic construct
  REGION 1..19: note = Self-cleaving polypeptide comprising 2A site
TLNFDLLKLAGDVESNPGP

SEQ ID NO: 97 - protein, 14 aa, synthetic construct
  REGION 1..14: note = Self-cleaving polypeptide comprising 2A site
LLKLAGDVESNPGP

SEQ ID NO: 98 - protein, 17 aa, synthetic construct
  REGION 1..17: note = Self-cleaving polypeptide comprising 2A site
NFDLLKLAGDVESNPGP

SEQ ID NO: 99 - protein, 20 aa, synthetic construct
  REGION 1..20: note = Self-cleaving polypeptide comprising 2A site
QLLNFDLLKLAGDVESNPGP

SEQ ID NO: 100 - protein, 24 aa, synthetic construct
  REGION 1..24: note = Self-cleaving polypeptide comprising 2A site
APVKQTLNFDLLKLAGDVESNPGP

SEQ ID NO: 101 - protein, 40 aa, synthetic construct
  REGION 1..40: note = Self-cleaving polypeptide comprising 2A site
VTELLYRMKRAETYCPRPLLAIHPTEARHKQKIVAPVKQT

SEQ ID NO: 102 - protein, 18 aa, synthetic construct
  REGION 1..18: note = Self-cleaving polypeptide comprising 2A site
LNFDLLKLAGDVESNPGP

SEQ ID NO: 103 - protein, 40 aa, synthetic construct
  REGION 1..40: note = Self-cleaving polypeptide comprising 2A site
LLAIHPTEARHKQKIVAPVKQTLNFDLLKLAGDVESNPGP

SEQ ID NO: 104 - protein, 33 aa, synthetic construct
  REGION 1..33: note = Self-cleaving polypeptide comprising 2A site
EARHKQKIVAPVKQTLNFDLLKLAGDVESNPGP

SEQ ID NO: 105 - DNA, 10 bp, synthetic construct
  misc_feature 1..10: note = Consensus Kozak sequence
  source 1..10: mol_type = other DNA
gccrccatgg

SEQ ID NO: 106 - protein, 8 aa, Homo sapiens
EQTEYATI

SEQ ID NO: 107 - DNA, 43 bp, Homo sapiens
  source 1..43: mol_type = unassigned DNA
tgagcagacggagtatgccaccattgtctttcctagcggaatg

SEQ ID NO: 108 - DNA, 43 bp, synthetic construct
  misc_feature 1..43: note = Made in Lab
  source 1..43: mol_type = other DNA
cattccgctaggaaagacaatggtggcatactccgtctgctca

SEQ ID NO: 109 - DNA, 22 bp, synthetic construct
  misc_feature 1..22: note = Made in Lab
  misc_feature 14..22: note = n is A, C, G or T
  source 1..22: mol_type = other DNA
aatggtggcatacnnnnnnnnn

SEQ ID NO: 110 - DNA, 22 bp, synthetic construct
  misc_feature 1..22: note = Made in Lab
  misc_feature 1..9: note = n is a, c, g, or t
  source 1..22: mol_type = other DNA
nnnnnnnnnatactccgtctgc

SEQ ID NO: 111 - DNA, 22 bp, synthetic construct
  misc_feature 1..22: note = Made in Lab
  source 1..22: mol_type = other DNA
aatggtggcatactccgtctgc

SEQ ID NO: 112 - DNA, 43 bp, Homo sapiens
  source 1..43: mol_type = unassigned DNA
attccgctaggaaagacaatggtggcatactccgtctgctcag

SEQ ID NO: 113 - DNA, 43 bp, synthetic construct
  misc_feature 1..43: note = Made in Lab
  source 1..43: mol_type = other DNA
atttcgttaggaaagataatggtggtatatttcgtttgtttag

SEQ ID NO: 114 - protein, 7 aa, Homo sapiens
MQIPQAP

SEQ ID NO: 115 - DNA, 44 bp, Homo sapiens
  source 1..44: mol_type = unassigned DNA
ctctggtggggctgctccaggcatgcagatcccacaggcgccct

SEQ ID NO: 116 - DNA, 44 bp, synthetic construct
  misc_feature 1..44: note = Made in Lab
  source 1..44: mol_type = other DNA
agggcgcctgtgggatctgcatccctggagcagccccaccagag

SEQ ID NO: 117 - protein, 8 aa, Homo sapiens
NGRDFHMS

SEQ ID NO: 118 - DNA, 43 bp, Homo sapiens
  source 1..43: mol_type = unassigned DNA
gtgtcacacaactgcccaacgggcgtgacttccacatgagcgt

SEQ ID NO: 119 - DNA, 43 bp, synthetic construct
  misc_feature 1..43: note = Made in Lab
  source 1..43: mol_type = other DNA
acgctcatgtggaagtcacgcccgttgggcagttgtgtgacac

SEQ ID NO: 120 - DNA, 32 bp, Homo sapiens
  source 1..32: mol_type = unassigned DNA
gctccaggcatgcagatcccacaggcgccctg

SEQ ID NO: 121 - DNA, 32 bp, synthetic construct
  misc_feature 1..32: note = made in lab
  source 1..32: mol_type = other DNA
actccaaacatacaaatcccacaaacacccta

SEQ ID NO: 122 - DNA, 31 bp, Homo sapiens
  source 1..31: mol_type = unassigned DNA
gcccaacgggcgtgacttccacatgagcgtg

SEQ ID NO: 123 - DNA, 31 bp, synthetic construct
  misc_feature 1..31: note = Made in Lab
  source 1..31: mol_type = other DNA
acccaacgaacgtaacttccacataaacgta